European Patent Specification EP 4 001 297 B1, published May 14, 2025. Title: CHIMERIC PAPILLOMAVIRUS L1 PROTEIN. Applicant: SinoCellTech Ltd. The sequence listing filed with the application follows.

SEQUENCE LISTING (156 sequences)

SEQ ID NO: 1 - protein, 469 aa, Homo sapiens
  0601 Amino acid sequence of HPV type 6 L1 protein aa 1-469
MWRPSDSTVYVPPPNPVSKVVATDAYVTRTNIFYHASSSRLLAVGHPYFSIKRANKTVVPKVSGYQYRVFKVVLPDPNKFALPDSSLFDPTTQRLVWACTGLEVGRGQPLGVGVSGHPFLNKYDDVENSGSGGNPGQDNRVNVGMDYKQTQLCMVGCAPPLGEHWGKGKQCTNTPVQAGDCPPLELITSVIQDGDMVDTGFGAMNFADLQTNKSDVPIDICGTTCKYPDYLQMAADPYGDRLFFFLRKEQMFARHFFNRAGEVGEPVPDTLIIKGSGNRTSVGSSIYVNTPSGSLVSSEAQLFNKPYWLQKAQGHNNGICWGNQLFVTVVDTTRSTNMTLCASVTTSSTYTNSDYKEYMRHVEEYDLQFIFQLCSITLSAEVMAYIHTMNPSVLEDWNFGLSPPPNGTLEDTYRYVQSQAITCQKPTPEKEKPDPYKNLSFWEVNLKEKFSSELDQYPLGRKFLLQSGY

SEQ ID NO: 2 - protein, 26 aa, Homo sapiens
  0602 Amino acid sequence of HPV type 33 L1 protein aa 474-499
KAKPKLKRAAPTSTRTSSAKRKKVKK

SEQ ID NO: 3 - protein, 495 aa, Artificial sequence
  0603 Amino acid sequence of chimeric HPV type 6 L1 protein
MWRPSDSTVYVPPPNPVSKVVATDAYVTRTNIFYHASSSRLLAVGHPYFSIKRANKTVVPKVSGYQYRVFKVVLPDPNKFALPDSSLFDPTTQRLVWACTGLEVGRGQPLGVGVSGHPFLNKYDDVENSGSGGNPGQDNRVNVGMDYKQTQLCMVGCAPPLGEHWGKGKQCTNTPVQAGDCPPLELITSVIQDGDMVDTGFGAMNFADLQTNKSDVPIDICGTTCKYPDYLQMAADPYGDRLFFFLRKEQMFARHFFNRAGEVGEPVPDTLIIKGSGNRTSVGSSIYVNTPSGSLVSSEAQLFNKPYWLQKAQGHNNGICWGNQLFVTVVDTTRSTNMTLCASVTTSSTYTNSDYKEYMRHVEEYDLQFIFQLCSITLSAEVMAYIHTMNPSVLEDWNFGLSPPPNGTLEDTYRYVQSQAITCQKPTPEKEKPDPYKNLSFWEVNLKEKFSSELDQYPLGRKFLLQSGYKAKPKLKRAAPTSTRTSSAKRKKVKK

SEQ ID NO: 4 - DNA, 1488 bp, Artificial sequence
  0604 Nucleotide sequence of chimeric HPV type 6 L1 protein
atgtggagaccatctgacagcacagtctatgtgcctcctccaaaccctgtgagcaaggtggtggctacagatgcctatgtgaccaggaccaacatcttctaccatgcctcctccagcagactgctggctgtgggacacccatacttcagcatcaagagggctaacaagacagtggtgccaaaggtgtctggctaccaatacagggtgttcaaggtggtgctgcctgacccaaacaagtttgccctgcctgactcctccctgtttgacccaaccacccagagactggtgtgggcttgtactggattggaggtgggcaggggacaaccactgggagtgggagtgtctggacacccattcctgaacaaatatgatgatgtggagaactctggctctggaggcaaccctggacaagacaacagggtgaatgtggggatggactacaagcagacccaactttgtatggtgggctgtgcccctccactgggagaacactggggcaagggcaagcagtgtaccaacacacctgtccaggctggagactgtcctccattggaactgattacctctgtgattcaggatggagatatggtggacacaggctttggagctatgaactttgctgacctccaaaccaacaagtctgatgtgccaattgacatctgtggcaccacttgtaaataccctgactacctccaaatggctgctgacccatatggagacagactgttcttcttcctgaggaaggaacagatgtttgccagacacttcttcaacagggctggagaggtgggagaacctgtgcctgacaccctgattatcaagggctctggcaacaggacctctgtgggctccagcatctatgtgaacacaccatctggctccctggtgtcctctgaggctcaacttttcaacaagccatactggctccaaaaggctcaaggacacaacaatggcatctgttggggcaaccaactttttgtgacagtggtggacaccaccaggagcaccaatatgaccctgtgtgcctctgtgaccacctccagcacctacaccaactctgactacaaggaatatatgaggcatgtggaggaatatgacctccaattcatcttccaactttgtagcatcaccctgtctgctgaggtgatggcttacatccacacaatgaacccatctgtgttggaggactggaactttggactgagccctcctccaaatggcaccttggaggacacctacagatatgtccagagccaggctatcacttgtcagaagccaacacctgagaaggagaagcctgacccatacaagaacctgtccttctgggaggtgaacctgaaagagaagttctcctctgaactggaccaatacccactgggcaggaagttcctgctccaatctggctacaaagccaagccaaaactgaaaagggctgccccaaccagcaccaggacctcctctgccaagaggaagaaggtgaagaagtaa

SEQ ID NO: 5 - DNA, 1522 bp, Artificial sequence
  0605 Synthetic HPV6 L1 gene
ctgggtaccatgtggagaccatctgacagcacagtctatgtgcctcctccaaaccctgtgagcaaggtggtggctacagatgcctatgtgaccaggaccaacatcttctaccatgcctcctccagcagactgctggctgtgggacacccatacttcagcatcaagagggctaacaagacagtggtgccaaaggtgtctggctaccaatacagggtgttcaaggtggtgctgcctgacccaaacaagtttgccctgcctgactcctccctgtttgacccaaccacccagagactggtgtgggcttgtactggattggaggtgggcaggggacaaccactgggagtgggagtgtctggacacccattcctgaacaaatatgatgatgtggagaactctggctctggaggcaaccctggacaagacaacagggtgaatgtggggatggactacaagcagacccaactttgtatggtgggctgtgcccctccactgggagaacactggggcaagggcaagcagtgtaccaacacacctgtccaggctggagactgtcctccattggaactgattacctctgtgattcaggatggagatatggtggacacaggctttggagctatgaactttgctgacctccaaaccaacaagtctgatgtgccaattgacatctgtggcaccacttgtaaataccctgactacctccaaatggctgctgacccatatggagacagactgttcttcttcctgaggaaggaacagatgtttgccagacacttcttcaacagggctggagaggtgggagaacctgtgcctgacaccctgattatcaagggctctggcaacaggacctctgtgggctccagcatctatgtgaacacaccatctggctccctggtgtcctctgaggctcaacttttcaacaagccatactggctccaaaaggctcaaggacacaacaatggcatctgttggggcaaccaactttttgtgacagtggtggacaccaccaggagcaccaatatgaccctgtgtgcctctgtgaccacctccagcacctacaccaactctgactacaaggaatatatgaggcatgtggaggaatatgacctccaattcatcttccaactttgtagcatcaccctgtctgctgaggtgatggcttacatccacacaatgaacccatctgtgttggaggactggaactttggactgagccctcctccaaatggcaccttggaggacacctacagatatgtccagagccaggctatcacttgtcagaagccaacacctgagaaggagaagcctgacccatacaagaacctgtccttctgggaggtgaacctgaaagagaagttctcctctgaactggaccaatacccactgggcaggaagttcctgctccaatctggctacaggggcaggtccagcatcaggacaggagtgaagagacctgctgtgagcaaggcatctgctgccccaaagaggaagagggctaagaccaagaggtaaactcgagctc

SEQ ID NO: 6 - DNA, 1519 bp, Artificial sequence
  0606 Synthetic HPV33 L1 gene
ctgggtaccatgagtgtgtggagaccatctgaggctacagtctacctgcctcctgtgcctgtgagcaaggtggtgagcacagatgaatatgtgagcaggaccagcatctactactatgctggctccagcagactgctggctgtgggacacccatacttcagcatcaagaacccaaccaatgccaagaaactgctggtgccaaaggtgtctggactccaatacagggtgttcagggtgagactgcctgacccaaacaagtttggctttcctgacacctccttctacaaccctgacacccagagactggtgtgggcttgtgtgggattggagattggcaggggacaaccactgggagtgggcatctctggacacccactgctgaacaagtttgatgacacagagacaggcaacaaataccctggacaacctggagcagacaacagggagtgtctgagtatggactacaagcagacccaactttgtctgctgggctgtaagcctccaacaggagaacactggggcaagggagtggcttgtaccaatgctgcccctgccaatgactgtcctccattggaactgataaacaccatcattgaggatggagatatggtggacacaggctttggctgtatggacttcaagaccctccaagccaacaagtctgatgtgccaattgacatctgtggcagcacttgtaaataccctgactacctgaaaatgacctctgaaccatatggagactccctgttcttcttcctgaggagggaacagatgtttgtgagacacttcttcaacagggctggcaccctgggagaggctgtgcctgatgacctctacatcaagggctctggcaccacagccagcatccagtcctctgccttctttccaacaccatctggcagtatggtgacctctgagagccaacttttcaacaagccatactggctccaaagggctcaaggacacaacaatggcatctgttggggcaaccaggtgtttgtgacagtggtggacaccaccaggagcaccaatatgaccctgtgtacccaggtgacctctgacagcacctacaagaatgagaacttcaaggaatacatcaggcatgtggaggaatatgacctccaatttgtgttccaactttgtaaggtgaccctgacagcagaggtgatgacctacatccatgctatgaaccctgacatcttggaggactggcagtttggactgacacctcctccatctgcctccctccaagacacctacaggtttgtgaccagccaggctatcacttgtcagaagacagtgcctccaaaggagaaggaggacccactgggcaaatacaccttctgggaggtggacctgaaagagaagttctctgctgacctggaccagtttccactgggcaggaagttcctgctccaagcaggactgaaagccaagccaaaactgaaaagggctgccccaaccagcaccaggacctcctctgccaagaggaagaaggtgaagaagtaaactcgagctc

SEQ ID NO: 7 - DNA, 35 bp, Artificial sequence
  0607 HPV6L1 F1
cttggtaccatgtggagaccatctgacagcacagt

SEQ ID NO: 8 - DNA, 36 bp, Artificial sequence
  0608 HPV6L1 R1
gcttggctttgtagccagattggagcaggaacttcc

SEQ ID NO: 9 - DNA, 1426 bp, Artificial sequence
  0609 HPV6L1 amplified sequence 1
cttggtaccatgtggagaccatctgacagcacagtctatgtgcctcctccaaaccctgtgagcaaggtggtggctacagatgcctatgtgaccaggaccaacatcttctaccatgcctcctccagcagactgctggctgtgggacacccatacttcagcatcaagagggctaacaagacagtggtgccaaaggtgtctggctaccaatacagggtgttcaaggtggtgctgcctgacccaaacaagtttgccctgcctgactcctccctgtttgacccaaccacccagagactggtgtgggcttgtactggattggaggtgggcaggggacaaccactgggagtgggagtgtctggacacccattcctgaacaaatatgatgatgtggagaactctggctctggaggcaaccctggacaagacaacagggtgaatgtggggatggactacaagcagacccaactttgtatggtgggctgtgcccctccactgggagaacactggggcaagggcaagcagtgtaccaacacacctgtccaggctggagactgtcctccattggaactgattacctctgtgattcaggatggagatatggtggacacaggctttggagctatgaactttgctgacctccaaaccaacaagtctgatgtgccaattgacatctgtggcaccacttgtaaataccctgactacctccaaatggctgctgacccatatggagacagactgttcttcttcctgaggaaggaacagatgtttgccagacacttcttcaacagggctggagaggtgggagaacctgtgcctgacaccctgattatcaagggctctggcaacaggacctctgtgggctccagcatctatgtgaacacaccatctggctccctggtgtcctctgaggctcaacttttcaacaagccatactggctccaaaaggctcaaggacacaacaatggcatctgttggggcaaccaactttttgtgacagtggtggacaccaccaggagcaccaatatgaccctgtgtgcctctgtgaccacctccagcacctacaccaactctgactacaaggaatatatgaggcatgtggaggaatatgacctccaattcatcttccaactttgtagcatcaccctgtctgctgaggtgatggcttacatccacacaatgaacccatctgtgttggaggactggaactttggactgagccctcctccaaatggcaccttggaggacacctacagatatgtccagagccaggctatcacttgtcagaagccaacacctgagaaggagaagcctgacccatacaagaacctgtccttctgggaggtgaacctgaaagagaagttctcctctgaactggaccaatacccactgggcaggaagttcctgctccaatctggctacaaagccaagc

SEQ ID NO: 10 - DNA, 35 bp, Artificial sequence
  0610 HPV6L1 F2
atctggctacaaagccaagccaaaactgaaaaggg

SEQ ID NO: 11 - DNA, 37 bp, Artificial sequence
  0611 HPV6L1 R2
ctgtctagatttacttcttcaccttcttcctcttggc

SEQ ID NO: 12 - DNA, 101 bp, Artificial sequence
  0612 HPV6L1 amplified sequence 2
atctggctacaaagccaagccaaaactgaaaagggctgccccaaccagcaccaggacctcctctgccaagaggaagaaggtgaagaagtaaatctagacag

SEQ ID NO: 13 - protein, 38 aa, Homo sapiens
  0613 Amino acid sequence of HPV type 59 L1 protein aa 471-508
LQLGARPKPTIGPRKRAAPAPTSTPSPKRVKRRKSSRK

SEQ ID NO: 14 - protein, 470 aa, Homo sapiens
  1101 Amino acid sequence of HPV type 11 L1 protein aa 1-470
MWRPSDSTVYVPPPNPVSKVVATDAYVKRTNIFYHASSSRLLAVGHPYYSIKKVNKTVVPKVSGYQYRVFKVVLPDPNKFALPDSSLFDPTTQRLVWACTGLEVGRGQPLGVGVSGHPLLNKYDDVENSGGYGGNPGQDNRVNVGMDYKQTQLCMVGCAPPLGEHWGKGTQCSNTSVQNGDCPPLELITSVIQDGDMVDTGFGAMNFADLQTNKSDVPLDICGTVCKYPDYLQMAADPYGDRLFFYLRKEQMFARHFFNRAGTVGEPVPDDLLVKGGNNRSSVASSIYVHTPSGSLVSSEAQLFNKPYWLQKAQGHNNGICWGNHLFVTVVDTTRSTNMTLCASVSKSATYTNSDYKEYMRHVEEFDLQFIFQLCSITLSAEVMAYIHTMNPSVLEDWNFGLSPPPNGTLEDTYRYVQSQAITCQKPTPEKEKQDPYKDMSFWEVNLKEKFSSELDQFPLGRKFLLQSGY

SEQ ID NO: 15 - protein, 26 aa, Homo sapiens
  1102 Amino acid sequence of HPV type 33 L1 protein aa 474-499
KAKPKLKRAAPTSTRTSSAKRKKVKK

SEQ ID NO: 16 - protein, 496 aa, Artificial sequence
  1103 Amino acid sequence of chimeric HPV type 11 L1 protein
MWRPSDSTVYVPPPNPVSKVVATDAYVKRTNIFYHASSSRLLAVGHPYYSIKKVNKTVVPKVSGYQYRVFKVVLPDPNKFALPDSSLFDPTTQRLVWACTGLEVGRGQPLGVGVSGHPLLNKYDDVENSGGYGGNPGQDNRVNVGMDYKQTQLCMVGCAPPLGEHWGKGTQCSNTSVQNGDCPPLELITSVIQDGDMVDTGFGAMNFADLQTNKSDVPLDICGTVCKYPDYLQMAADPYGDRLFFYLRKEQMFARHFFNRAGTVGEPVPDDLLVKGGNNRSSVASSIYVHTPSGSLVSSEAQLFNKPYWLQKAQGHNNGICWGNHLFVTVVDTTRSTNMTLCASVSKSATYTNSDYKEYMRHVEEFDLQFIFQLCSITLSAEVMAYIHTMNPSVLEDWNFGLSPPPNGTLEDTYRYVQSQAITCQKPTPEKEKQDPYKDMSFWEVNLKEKFSSELDQFPLGRKFLLQSGYKAKPKLKRAAPTSTRTSSAKRKKVKK

SEQ ID NO: 17 - DNA, 1492 bp, Artificial sequence
  1104 Nucleotide sequence of chimeric HPV type 11 L1 protein
atgtggagaccatctgacagcacagtctatgtgcctcctccaaaccctgtgagcaaggtggtggctacagatgcctatgtgaagaggaccaacatcttctaccatgcctcctccagcagactgctggctgtgggacacccatactacagcatcaagaaggtgaacaagacagtggtgccaaaggtgtctggctaccaatacagggtgttcaaggtggtgctgcctgacccaaacaagtttgccctgcctgactcctccctgtttgacccaaccacccagagactggtgtgggcttgtactggattggaggtgggcaggggacaaccactgggagtgggagtgtctggacacccactgctgaacaaatatgatgatgtggagaactctggaggctatggaggcaaccctggacaagacaacagggtgaatgtggggatggactacaagcagacccaactttgtatggtgggctgtgcccctccactgggagaacactggggcaagggcacccagtgtagcaacacctctgtccagaatggagactgtcctccattggaactgattacctctgtgattcaggatggagatatggtggacacaggctttggagctatgaactttgctgacctccaaaccaacaagtctgatgtgccactggacatctgtggcacagtgtgtaaataccctgactacctccaaatggctgctgacccatatggagacagactgttcttctacctgaggaaggaacagatgtttgccagacacttcttcaacagggctggcacagtgggagaacctgtgcctgatgacctgctggtgaagggaggcaacaacaggtcctctgtggcatccagcatctatgtgcatacaccatctggctccctggtgtcctctgaggctcaacttttcaacaagccatactggctccaaaaggctcaaggacacaacaatggcatctgttggggcaaccacctgtttgtgacagtggtggacaccaccaggagcaccaatatgaccctgtgtgcctctgtgagcaagtctgccacctacaccaactctgactacaaggaatatatgaggcatgtggaggagtttgacctccaattcatcttccaactttgtagcatcaccctgtctgctgaggtgatggcttacatccacacaatgaacccatctgtgttggaggactggaactttggactgagccctcctccaaatggcaccttggaggacacctacagatatgtccagagccaggctatcacttgtcagaagccaacacctgagaaggagaagcaggacccatacaaggatatgagtttctgggaggtgaacctgaaagagaagttctcctctgaactggaccagtttccactgggcaggaagttcctgctccaatctggctacaaagccaagccaaaactgaaaagggctgccccaaccagcaccaggacctcctctgccaagaggaagaaggtgaagaagtaaa

SEQ ID NO: 18 - DNA, 1525 bp, Artificial sequence
  1105 Synthetic HPV11 L1 gene
ctgggtaccatgtggagaccatctgacagcacagtctatgtgcctcctccaaaccctgtgagcaaggtggtggctacagatgcctatgtgaagaggaccaacatcttctaccatgcctcctccagcagactgctggctgtgggacacccatactacagcatcaagaaggtgaacaagacagtggtgccaaaggtgtctggctaccaatacagggtgttcaaggtggtgctgcctgacccaaacaagtttgccctgcctgactcctccctgtttgacccaaccacccagagactggtgtgggcttgtactggattggaggtgggcaggggacaaccactgggagtgggagtgtctggacacccactgctgaacaaatatgatgatgtggagaactctggaggctatggaggcaaccctggacaagacaacagggtgaatgtggggatggactacaagcagacccaactttgtatggtgggctgtgcccctccactgggagaacactggggcaagggcacccagtgtagcaacacctctgtccagaatggagactgtcctccattggaactgattacctctgtgattcaggatggagatatggtggacacaggctttggagctatgaactttgctgacctccaaaccaacaagtctgatgtgccactggacatctgtggcacagtgtgtaaataccctgactacctccaaatggctgctgacccatatggagacagactgttcttctacctgaggaaggaacagatgtttgccagacacttcttcaacagggctggcacagtgggagaacctgtgcctgatgacctgctggtgaagggaggcaacaacaggtcctctgtggcatccagcatctatgtgcatacaccatctggctccctggtgtcctctgaggctcaacttttcaacaagccatactggctccaaaaggctcaaggacacaacaatggcatctgttggggcaaccacctgtttgtgacagtggtggacaccaccaggagcaccaatatgaccctgtgtgcctctgtgagcaagtctgccacctacaccaactctgactacaaggaatatatgaggcatgtggaggagtttgacctccaattcatcttccaactttgtagcatcaccctgtctgctgaggtgatggcttacatccacacaatgaacccatctgtgttggaggactggaactttggactgagccctcctccaaatggcaccttggaggacacctacagatatgtccagagccaggctatcacttgtcagaagccaacacctgagaaggagaagcaggacccatacaaggatatgagtttctgggaggtgaacctgaaagagaagttctcctctgaactggaccagtttccactgggcaggaagttcctgctccaatctggctacaggggcaggacctctgccaggacaggcatcaagagacctgctgtgagcaagccaagcacagccccaaagaggaagaggaccaagaccaagaagtaaactcgagctc

SEQ ID NO: 19 - DNA, 1519 bp, Artificial sequence; identical to SEQ ID NO: 6
  1106 Synthetic HPV33 L1 gene

SEQ ID NO: 20 - DNA, 35 bp, Artificial sequence; identical to SEQ ID NO: 7
  1107 HPV11L1 F1

SEQ ID NO: 21 - DNA, 36 bp, Artificial sequence; identical to SEQ ID NO: 8
  1108 HPV11L1 R1

SEQ ID NO: 22 - DNA, 1429 bp, Artificial sequence
  1109 HPV11L1 amplified sequence 1
cttggtaccatgtggagaccatctgacagcacagtctatgtgcctcctccaaaccctgtgagcaaggtggtggctacagatgcctatgtgaagaggaccaacatcttctaccatgcctcctccagcagactgctggctgtgggacacccatactacagcatcaagaaggtgaacaagacagtggtgccaaaggtgtctggctaccaatacagggtgttcaaggtggtgctgcctgacccaaacaagtttgccctgcctgactcctccctgtttgacccaaccacccagagactggtgtgggcttgtactggattggaggtgggcaggggacaaccactgggagtgggagtgtctggacacccactgctgaacaaatatgatgatgtggagaactctggaggctatggaggcaaccctggacaagacaacagggtgaatgtggggatggactacaagcagacccaactttgtatggtgggctgtgcccctccactgggagaacactggggcaagggcacccagtgtagcaacacctctgtccagaatggagactgtcctccattggaactgattacctctgtgattcaggatggagatatggtggacacaggctttggagctatgaactttgctgacctccaaaccaacaagtctgatgtgccactggacatctgtggcacagtgtgtaaataccctgactacctccaaatggctgctgacccatatggagacagactgttcttctacctgaggaaggaacagatgtttgccagacacttcttcaacagggctggcacagtgggagaacctgtgcctgatgacctgctggtgaagggaggcaacaacaggtcctctgtggcatccagcatctatgtgcatacaccatctggctccctggtgtcctctgaggctcaacttttcaacaagccatactggctccaaaaggctcaaggacacaacaatggcatctgttggggcaaccacctgtttgtgacagtggtggacaccaccaggagcaccaatatgaccctgtgtgcctctgtgagcaagtctgccacctacaccaactctgactacaaggaatatatgaggcatgtggaggagtttgacctccaattcatcttccaactttgtagcatcaccctgtctgctgaggtgatggcttacatccacacaatgaacccatctgtgttggaggactggaactttggactgagccctcctccaaatggcaccttggaggacacctacagatatgtccagagccaggctatcacttgtcagaagccaacacctgagaaggagaagcaggacccatacaaggatatgagtttctgggaggtgaacctgaaagagaagttctcctctgaactggaccagtttccactgggcaggaagttcctgctccaatctggctacaaagccaagc

SEQ ID NO: 23 - DNA, 35 bp, Artificial sequence; identical to SEQ ID NO: 10
  1110 HPV11L1 F2

SEQ ID NO: 24 - DNA, 37 bp, Artificial sequence; identical to SEQ ID NO: 11
  1111 HPV11L1 R2

SEQ ID NO: 25 - DNA, 101 bp, Artificial sequence; identical to SEQ ID NO: 12
  1112 HPV11L1 amplified sequence 2

SEQ ID NO: 26 - protein, 38 aa, Homo sapiens; identical to SEQ ID NO: 13
  1113 Amino acid sequence of HPV type 59 L1 protein aa 471-508

SEQ ID NO: 27 - protein, 474 aa, Homo sapiens
  1601 Amino acid sequence of HPV type 16 L1 protein aa 1-474
MSLWLPSEATVYLPPVPVSKVVSTDEYVARTNIYYHAGTSRLLAVGHPYFPIKKPNNNKILVPKVSGLQYRVFRIHLPDPNKFGFPDTSFYNPDTQRLVWACVGVEVGRGQPLGVGISGHPLLNKLDDTENASAYAANAGVDNRECISMDYKQTQLCLIGCKPPIGEHWGKGSPCTNVAVNPGDCPPLELINTVIQDGDMVDTGFGAMDFTTLQANKSEVPLDICTSICKYPDYIKMVSEPYGDSLFFYLRREQMFVRHLFNRAGAVGENVPDDLYIKGSGSTANLASSNYFPTPSGSMVTSDAQIFNKPYWLQRAQGHNNGICWGNQLFVTVVDTTRSTNMSLCAAISTSETTYKNTNFKEYLRHGEEYDLQFIFQLCKITLTADVMTYIHSMNSTILEDWNFGLQPPPGGTLEDTYRFVTSQAIACQKHTPPAPKEDPLKKYTFWEVNLKEKFSADLDQFPLGRKFLLQAGL

SEQ ID NO: 28 - protein, 26 aa, Homo sapiens
  1602 Amino acid sequence of HPV type 33 L1 protein aa 474-499
KAKPKLKRAAPTSTRTSSAKRKKVKK

SEQ ID NO: 29 - protein, 500 aa, Artificial sequence
  1603 Amino acid sequence of chimeric HPV type 16 L1 protein
MSLWLPSEATVYLPPVPVSKVVSTDEYVARTNIYYHAGTSRLLAVGHPYFPIKKPNNNKILVPKVSGLQYRVFRIHLPDPNKFGFPDTSFYNPDTQRLVWACVGVEVGRGQPLGVGISGHPLLNKLDDTENASAYAANAGVDNRECISMDYKQTQLCLIGCKPPIGEHWGKGSPCTNVAVNPGDCPPLELINTVIQDGDMVDTGFGAMDFTTLQANKSEVPLDICTSICKYPDYIKMVSEPYGDSLFFYLRREQMFVRHLFNRAGAVGENVPDDLYIKGSGSTANLASSNYFPTPSGSMVTSDAQIFNKPYWLQRAQGHNNGICWGNQLFVTVVDTTRSTNMSLCAAISTSETTYKNTNFKEYLRHGEEYDLQFIFQLCKITLTADVMTYIHSMNSTILEDWNFGLQPPPGGTLEDTYRFVTSQAIACQKHTPPAPKEDPLKKYTFWEVNLKEKFSADLDQFPLGRKFLLQAGLKAKPKLKRAAPTSTRTSSAKRKKVKK

SEQ ID NO: 30 - DNA, 1504 bp, Artificial sequence
  1604 Nucleotide sequence of chimeric HPV type 16 L1 protein
atgagtctgtggctgccatctgaggctacagtctacctgcctcctgtgcctgtgagcaaggtggtgagcacagatgaatatgtggcaaggaccaacatctactaccatgctggcaccagcagactgctggctgtgggacacccatactttccaatcaagaagccaaacaacaacaagattctggtgccaaaggtgtctggactccaatacagggtgttcaggattcacctgcctgacccaaacaagtttggctttcctgacacctccttctacaaccctgacacccagagactggtgtgggcttgtgtgggagtggaggtgggcaggggacaaccactgggagtgggcatctctggacacccactgctgaacaaactggatgacacagagaatgcctctgcctatgctgccaatgctggagtggacaacagggagtgtatcagtatggactacaagcagacccaactttgtctgattggctgtaagcctccaattggagaacactggggcaagggcagcccatgtaccaatgtggctgtgaaccctggagactgtcctccattggaactgataaacacagtgattcaggatggagatatggtggacacaggctttggagctatggacttcaccaccctccaagccaacaagtctgaggtgccactggacatctgtaccagcatctgtaaataccctgactacatcaagatggtgtctgaaccatatggagactccctgttcttctacctgaggagggaacagatgtttgtgagacacctgttcaacagggctggagcagtgggagagaatgtgcctgatgacctctacatcaagggctctggcagcacagccaacctggcatccagcaactactttccaacaccatctggcagtatggtgacctctgatgcccagattttcaacaagccatactggctccaaagggctcaaggacacaacaatggcatctgttggggcaaccaactttttgtgacagtggtggacaccaccaggagcaccaatatgagtctgtgtgctgccatcagcacctctgagaccacctacaagaacaccaacttcaaggaatacctgagacatggagaggaatatgacctccaattcatcttccaactttgtaagattaccctgacagcagatgtgatgacctacatccacagtatgaacagcaccatcttggaggactggaactttggactccaacctcctcctggaggcaccttggaggacacctacaggtttgtgaccagccaggctattgcctgtcagaaacacacacctcctgccccaaaggaggacccactgaaaaaatacaccttctgggaggtgaacctgaaagagaagttctctgctgacctggaccagtttccactgggcaggaagttcctgctccaagcaggactgaaagccaagccaaaactgaaaagggctgccccaaccagcaccaggacctcctctgccaagaggaagaaggtgaagaagtaaa

SEQ ID NO: 31 - DNA, 1537 bp, Artificial sequence
  1605 Synthetic HPV16 L1 gene
ctgggtaccatgagtctgtggctgccatctgaggctacagtctacctgcctcctgtgcctgtgagcaaggtggtgagcacagatgaatatgtggcaaggaccaacatctactaccatgctggcaccagcagactgctggctgtgggacacccatactttccaatcaagaagccaaacaacaacaagattctggtgccaaaggtgtctggactccaatacagggtgttcaggattcacctgcctgacccaaacaagtttggctttcctgacacctccttctacaaccctgacacccagagactggtgtgggcttgtgtgggagtggaggtgggcaggggacaaccactgggagtgggcatctctggacacccactgctgaacaaactggatgacacagagaatgcctctgcctatgctgccaatgctggagtggacaacagggagtgtatcagtatggactacaagcagacccaactttgtctgattggctgtaagcctccaattggagaacactggggcaagggcagcccatgtaccaatgtggctgtgaaccctggagactgtcctccattggaactgataaacacagtgattcaggatggagatatggtggacacaggctttggagctatggacttcaccaccctccaagccaacaagtctgaggtgccactggacatctgtaccagcatctgtaaataccctgactacatcaagatggtgtctgaaccatatggagactccctgttcttctacctgaggagggaacagatgtttgtgagacacctgttcaacagggctggagcagtgggagagaatgtgcctgatgacctctacatcaagggctctggcagcacagccaacctggcatccagcaactactttccaacaccatctggcagtatggtgacctctgatgcccagattttcaacaagccatactggctccaaagggctcaaggacacaacaatggcatctgttggggcaaccaactttttgtgacagtggtggacaccaccaggagcaccaatatgagtctgtgtgctgccatcagcacctctgagaccacctacaagaacaccaacttcaaggaatacctgagacatggagaggaatatgacctccaattcatcttccaactttgtaagattaccctgacagcagatgtgatgacctacatccacagtatgaacagcaccatcttggaggactggaactttggactccaacctcctcctggaggcaccttggaggacacctacaggtttgtgaccagccaggctattgcctgtcagaaacacacacctcctgccccaaaggaggacccactgaaaaaatacaccttctgggaggtgaacctgaaagagaagttctctgctgacctggaccagtttccactgggcaggaagttcctgctccaagcaggactgaaagccaagccaaagttcaccctgggcaagaggaaggctacaccaaccacctccagcaccagcaccacagccaagaggaagaagaggaaactgtaaactcgagctc

SEQ ID NO: 32 - DNA, 1519 bp, Artificial sequence; identical to SEQ ID NO: 6
  1606 Synthetic HPV33 L1 gene

SEQ ID NO: 33 - DNA, 34 bp, Artificial sequence
  1607 HPV16L1 F1
cttggtaccatgagtctgtggctgccatctgagg

SEQ ID NO: 34 - DNA, 36 bp, Artificial sequence
  1608 HPV16L1 R1
gcttggctttcagtcctgcttggagcaggaacttcc

SEQ ID NO: 35 - DNA, 1441 bp, Artificial sequence
  1609 HPV16L1 amplified sequence 1
cttggtaccatgagtctgtggctgccatctgaggctacagtctacctgcctcctgtgcctgtgagcaaggtggtgagcacagatgaatatgtggcaaggaccaacatctactaccatgctggcaccagcagactgctggctgtgggacacccatactttccaatcaagaagccaaacaacaacaagattctggtgccaaaggtgtctggactccaatacagggtgttcaggattcacctgcctgacccaaacaagtttggctttcctgacacctccttctacaaccctgacacccagagactggtgtgggcttgtgtgggagtggaggtgggcaggggacaaccactgggagtgggcatctctggacacccactgctgaacaaactggatgacacagagaatgcctctgcctatgctgccaatgctggagtggacaacagggagtgtatcagtatggactacaagcagacccaactttgtctgattggctgtaagcctccaattggagaacactggggcaagggcagcccatgtaccaatgtggctgtgaaccctggagactgtcctccattggaactgataaacacagtgattcaggatggagatatggtggacacaggctttggagctatggacttcaccaccctccaagccaacaagtctgaggtgccactggacatctgtaccagcatctgtaaataccctgactacatcaagatggtgtctgaaccatatggagactccctgttcttctacctgaggagggaacagatgtttgtgagacacctgttcaacagggctggagcagtgggagagaatgtgcctgatgacctctacatcaagggctctggcagcacagccaacctggcatccagcaactactttccaacaccatctggcagtatggtgacctctgatgcccagattttcaacaagccatactggctccaaagggctcaaggacacaacaatggcatctgttggggcaaccaactttttgtgacagtggtggacaccaccaggagcaccaatatgagtctgtgtgctgccatcagcacctctgagaccacctacaagaacaccaacttcaaggaatacctgagacatggagaggaatatgacctccaattcatcttccaactttgtaagattaccctgacagcagatgtgatgacctacatccacagtatgaacagcaccatcttggaggactggaactttggactccaacctcctcctggaggcaccttggaggacacctacaggtttgtgaccagccaggctattgcctgtcagaaacacacacctcctgccccaaaggaggacccactgaaaaaatacaccttctgggaggtgaacctgaaagagaagttctctgctgacctggaccagtttccactgggcaggaagttcctgctccaagcaggactgaaagccaagc

SEQ ID NO: 36 - DNA, 35 bp, Artificial sequence
  1610 HPV16L1 F2
agcaggactgaaagccaagccaaaactgaaaaggg

SEQ ID NO: 37 - DNA, 36 bp, Artificial sequence
  1611 HPV16L1 R2
ctgtctagatttacttcttcaccttcttcctcttgg

SEQ ID NO: 38 - DNA, 101 bp, Artificial sequence
  1612 HPV16L1 amplified sequence 2
agcaggactgaaagccaagccaaaactgaaaagggctgccccaaccagcaccaggacctcctctgccaagaggaagaaggtgaagaagtaaatctagacag

SEQ ID NO: 39 - protein, 38 aa, Homo sapiens; identical to SEQ ID NO: 13
  1613 Amino acid sequence of HPV type 59 L1 protein aa 471-508

SEQ ID NO: 40 - protein, 470 aa, Homo sapiens
  1801 Amino acid sequence of HPV type 18 L1 protein aa 1-470
MALWRPSDNTVYLPPPSVARVVNTDDYVTRTSIFYHAGSSRLLTVGNPYFRVPAGGGNKQDIPKVSAYQYRVFRVQLPDPNKFGLPDTSIYNPETQRLVWACAGVEIGRGQPLGVGLSGHPFYNKLDDTESSHAATSNVSEDVRDNVSVDYKQTQLCILGCAPAIGEHWAKGTACKSRPLSQGDCPPLELKNTVLEDGDMVDTGYGAMDFSTLQDTKCEVPLDICQSICKYPDYLQMSADPYGDSMFFCLRREQLFARHFWNRAGTMGDTVPQSLYIKGTGMRASPGSCVYSPSPSGSIVTSDSQLFNKPYWLHKAQGHNNGVCWHNQLFVTVVDTTRSTNLTICASTQSPVPGQYDATKFKQYSRHVEEYDLQFIFQLCTITLTADVMSYIHSMNSSILEDWNFGVPPPPTTSLVDTYRFVQSVAITCQKDAAPAENKDPYDKLKFWNVDLKEKFSLDLDQYPLGRKFL

SEQ ID NO: 41 - protein, 26 aa, Homo sapiens
  1802 Amino acid sequence of HPV type 33 L1 protein aa 474-499
KAKPKLKRAAPTSTRTSSAKRKKVKK

SEQ ID NO: 42 - protein, 496 aa, Artificial sequence
  1803 Amino acid sequence of chimeric HPV type 18 L1 protein
MALWRPSDNTVYLPPPSVARVVNTDDYVTRTSIFYHAGSSRLLTVGNPYFRVPAGGGNKQDIPKVSAYQYRVFRVQLPDPNKFGLPDTSIYNPETQRLVWACAGVEIGRGQPLGVGLSGHPFYNKLDDTESSHAATSNVSEDVRDNVSVDYKQTQLCILGCAPAIGEHWAKGTACKSRPLSQGDCPPLELKNTVLEDGDMVDTGYGAMDFSTLQDTKCEVPLDICQSICKYPDYLQMSADPYGDSMFFCLRREQLFARHFWNRAGTMGDTVPQSLYIKGTGMRASPGSCVYSPSPSGSIVTSDSQLFNKPYWLHKAQGHNNGVCWHNQLFVTVVDTTRSTNLTICASTQSPVPGQYDATKFKQYSRHVEEYDLQFIFQLCTITLTADVMSYIHSMNSSILEDWNFGVPPPPTTSLVDTYRFVQSVAITCQKDAAPAENKDPYDKLKFWNVDLKEKFSLDLDQYPLGRKFLKAKPKLKRAAPTSTRTSSAKRKKVKK

SEQ ID NO: 43 - DNA, 1492 bp, Artificial sequence
  1804 Nucleotide sequence of chimeric HPV type 18 L1 protein
atggccctctggagaccatccgataacacagtgtacttgcccccacccagcgtcgcccgggtggtgaacacagacgactacgtcaccagaacctcaatcttctaccacgccgggtccagccggctgctgaccgtgggcaacccctacttccgcgtgcccgccggcggcggaaacaaacaagacatccccaaagtcagcgcctatcagtaccgggtgttccgcgtccaactgcccgatcccaacaagttcggcctgcccgacacctccatctacaaccccgagacccagaggctggtctgggcttgcgccggcgtcgagatcgggaggggccaacccctgggcgtggggttgtccggccaccccttctacaacaagctggacgataccgagtccagccacgcagcaaccagcaacgtctccgaagatgtgcgcgataacgtcagcgtggactacaaacaaacccaactgtgcatcctgggatgcgcacccgccatcggcgagcattgggccaaggggaccgcctgcaagagcaggcccctgagccaaggggactgtccacccctggagttgaagaataccgtgctcgaggacggcgacatggtggacaccggctacggcgctatggatttctccaccctccaggacaccaagtgcgaagtgcccctcgacatctgccaaagcatctgcaagtaccccgactacctccagatgagcgccgacccctacggcgacagcatgttcttctgtctcagaagggaacaattgttcgcccgccacttctggaaccgggccggcacaatgggagatacagtcccccagagcctgtacatcaaggggaccggaatgagggccagccccgggtcctgcgtctacagcccaagcccctccgggagcatcgtcacaagcgatagccaactcttcaacaagccctactggctccacaaagcccaaggccacaataacggggtgtgttggcacaaccagctgttcgtgaccgtcgtggacacaaccaggtccacaaacctgaccatctgcgccagcacccaaagccccgtgcccggccagtacgacgccacaaagttcaaacaatactctcggcacgtggaagagtacgacctccaattcatcttccaactctgcaccatcaccctcaccgccgacgtgatgagctacatccactccatgaactcctccatcctggaagactggaatttcggcgtgccaccaccccctaccacctccctcgtcgacacctacagattcgtgcagagcgtggccatcacatgccagaaagacgccgcccccgccgagaacaaagacccatacgacaaactgaaattctggaacgtcgacctgaaagagaaattcagcctggatctggaccagtacccattgggcaggaagttcctcaaagccaagccaaaactgaaaagggctgccccaaccagcaccaggacctcctctgccaagaggaagaaggtgaagaagtaaa

SEQ ID NO: 44 - DNA, 1543 bp, Artificial sequence
  1805 Synthetic HPV18 L1 gene
ctgggtaccatggccctctggagaccatccgataacacagtgtacttgcccccacccagcgtcgcccgggtggtgaacacagacgactacgtcaccagaacctcaatcttctaccacgccgggtccagccggctgctgaccgtgggcaacccctacttccgcgtgcccgccggcggcggaaacaaacaagacatccccaaagtcagcgcctatcagtaccgggtgttccgcgtccaactgcccgatcccaacaagttcggcctgcccgacacctccatctacaaccccgagacccagaggctggtctgggcttgcgccggcgtcgagatcgggaggggccaacccctgggcgtggggttgtccggccaccccttctacaacaagctggacgataccgagtccagccacgcagcaaccagcaacgtctccgaagatgtgcgcgataacgtcagcgtggactacaaacaaacccaactgtgcatcctgggatgcgcacccgccatcggcgagcattgggccaaggggaccgcctgcaagagcaggcccctgagccaaggggactgtccacccctggagttgaagaataccgtgctcgaggacggcgacatggtggacaccggctacggcgctatggatttctccaccctccaggacaccaagtgcgaagtgcccctcgacatctgccaaagcatctgcaagtaccccgactacctccagatgagcgccgacccctacggcgacagcatgttcttctgtctcagaagggaacaattgttcgcccgccacttctggaaccgggccggcacaatgggagatacagtcccccagagcctgtacatcaaggggaccggaatgagggccagccccgggtcctgcgtctacagcccaagcccctccgggagcatcgtcacaagcgatagccaactcttcaacaagccctactggctccacaaagcccaaggccacaataacggggtgtgttggcacaaccagctgttcgtgaccgtcgtggacacaaccaggtccacaaacctgaccatctgcgccagcacccaaagccccgtgcccggccagtacgacgccacaaagttcaaacaatactctcggcacgtggaagagtacgacctccaattcatcttccaactctgcaccatcaccctcaccgccgacgtgatgagctacatccactccatgaactcctccatcctggaagactggaatttcggcgtgccaccaccccctaccacctccctcgtcgacacctacagattcgtgcagagcgtggccatcacatgccagaaagacgccgcccccgccgagaacaaagacccatacgacaaactgaaattctggaacgtcgacctgaaagagaaattcagcctggatctggaccagtacccattgggcaggaagttcctcgtgcaagccggcctcaggagaaaaccaacaatcgggcccaggaagaggagcgcccccagcgcaaccaccagcagcaagcccgcaaaaagggtcagagtgagggcacgcaaataaactcgagctc

SEQ ID NO: 45 - DNA, 1519 bp, Artificial sequence; identical to SEQ ID NO: 6
  1806 Synthetic HPV33 L1 gene

SEQ ID NO: 46 - DNA, 34 bp, Artificial sequence
  1807 HPV18L1 F1
cttggtaccatggccctctggagaccatccgata

SEQ ID NO: 47 - DNA, 35 bp, Artificial sequence
  1808 HPV18L1 R1
gcttggctttgaggaacttcctgcccaatgggtac

SEQ ID NO: 48 - DNA, 1429 bp, Artificial sequence
  1809 HPV18L1 amplified sequence 1
cttggtaccatggccctctggagaccatccgataacacagtgtacttgcccccacccagcgtcgcccgggtggtgaacacagacgactacgtcaccagaacctcaatcttctaccacgccgggtccagccggctgctgaccgtgggcaacccctacttccgcgtgcccgccggcggcggaaacaaacaagacatccccaaagtcagcgcctatcagtaccgggtgttccgcgtccaactgcccgatcccaacaagttcggcctgcccgacacctccatctacaaccccgagacccagaggctggtctgggcttgcgccggcgtcgagatcgggaggggccaacccctgggcgtggggttgtccggccaccccttctacaacaagctggacgataccgagtccagccacgcagcaaccagcaacgtctccgaagatgtgcgcgataacgtcagcgtggactacaaacaaacccaactgtgcatcctgggatgcgcacccgccatcggcgagcattgggccaaggggaccgcctgcaagagcaggcccctgagccaaggggactgtccacccctggagttgaagaataccgtgctcgaggacggcgacatggtggacaccggctacggcgctatggatttctccaccctccaggacaccaagtgcgaagtgcccctcgacatctgccaaagcatctgcaagtaccccgactacctccagatgagcgccgacccctacggcgacagcatgttcttctgtctcagaagggaacaattgttcgcccgccacttctggaaccgggccggcacaatgggagatacagtcccccagagcctgtacatcaaggggaccggaatgagggccagccccgggtcctgcgtctacagcccaagcccctccgggagcatcgtcacaagcgatagccaactcttcaacaagccctactggctccacaaagcccaaggccacaataacggggtgtgttggcacaaccagctgttcgtgaccgtcgtggacacaaccaggtccacaaacctgaccatctgcgccagcacccaaagccccgtgcccggccagtacgacgccacaaagttcaaacaatactctcggcacgtggaagagtacgacctccaattcatcttccaactctgcaccatcaccctcaccgccgacgtgatgagctacatccactccatgaactcctccatcctggaagactggaatttcggcgtgccaccaccccctaccacctccctcgtcgacacctacagattcgtgcagagcgtggccatcacatgccagaaagacgccgcccccgccgagaacaaagacccatacgacaaactgaaattctggaacgtcgacctgaaagagaaattcagcctggatctggaccagtacccattgggcaggaagttcctcaaagccaagc

SEQ ID NO: 49 - DNA, 35 bp, Artificial sequence
  1810 HPV18L1 F2
gaagttcctcaaagccaagccaaaactgaaaaggg

SEQ ID NO: 50 - DNA, 36 bp, Artificial sequence; identical to SEQ ID NO: 37
  1811 HPV18L1 R2

SEQ ID NO: 51 - DNA, 101 bp, Artificial sequence
  1812 HPV18L1 amplified sequence 2
gaagttcctcaaagccaagccaaaactgaaaagggctgccccaaccagcaccaggacctcctctgccaagaggaagaaggtgaagaagtaaatctagacag

SEQ ID NO: 52 - protein, 38 aa, Homo sapiens; identical to SEQ ID NO: 13
  1813 Amino acid sequence of HPV type 59 L1 protein aa 471-508

SEQ ID NO: 53 - protein, 475 aa, Homo sapiens
  3101 Amino acid sequence of HPV type 31 L1 protein aa 1-475
MSLWRPSEATVYLPPVPVSKVVSTDEYVTRTNIYYHAGSARLLTVGHPYYSIPKSDNPKKIVVPKVSGLQYRVFRVRLPDPNKFGFPDTSFYNPETQRLVWACVGLEVGRGQPLGVGISGHPLLNKFDDTENSNRYAGGPGTDNRECISMDYKQTQLCLLGCKPPIGEHWGKGSPCSNNAITPGDCPPLELKNSVIQDGDMVDTGFGAMDFTALQDTKSNVPLDICNSICKYPDYLKMVAEPYGDTLFFYLRREQMFVRHFFNRSGTVGESVPTDLYIKGSGSTATLANSTYFPTPSGSMVTSDAQIFNKPYWMQRAQGHNNGICWGNQLFVTVVDTTRSTNMSVCAAIANSDTTFKSSNFKEYLRHGEEFDLQFIFQLCKITLSADIMTYIHSMNPAILEDWNFGLTTPPSGSLEDTYRFVTSQAITCQKSAPQKPKEDPFKDYVFWEVNLKEKFSADLDQFPLGRKFLLQAGY

SEQ ID NO: 54 - protein, 26 aa, Homo sapiens
  3102 Amino acid sequence of HPV type 33 L1 protein aa 474-499
KAKPKLKRAAPTSTRTSSAKRKKVKK

SEQ ID NO: 55 - protein, 501 aa, Artificial sequence
  3103 Amino acid sequence of chimeric HPV type 31 L1 protein
MSLWRPSEATVYLPPVPVSKVVSTDEYVTRTNIYYHAGSARLLTVGHPYYSIPKSDNPKKIVVPKVSGLQYRVFRVRLPDPNKFGFPDTSFYNPETQRLVWACVGLEVGRGQPLGVGISGHPLLNKFDDTENSNRYAGGPGTDNRECISMDYKQTQLCLLGCKPPIGEHWGKGSPCSNNAITPGDCPPLELKNSVIQDGDMVDTGFGAMDFTALQDTKSNVPLDICNSICKYPDYLKMVAEPYGDTLFFYLRREQMFVRHFFNRSGTVGESVPTDLYIKGSGSTATLANSTYFPTPSGSMVTSDAQIFNKPYWMQRAQGHNNGICWGNQLFVTVVDTTRSTNMSVCAAIANSDTTFKSSNFKEYLRHGEEFDLQFIFQLCKITLSADIMTYIHSMNPAILEDWNFGLTTPPSGSLEDTYRFVTSQAITCQKSAPQKPKEDPFKDYVFWEVNLKEKFSADLDQFPLGRKFLLQAGYKAKPKLKRAAPTSTRTSSAKRKKVKK

SEQ ID NO: 56 - DNA, 1507 bp, Artificial sequence
  3104 Nucleotide sequence of chimeric HPV type 31 L1 protein
atgagcctgtggaggcccagcgaggccaccgtgtacctgccccccgtgcccgtgagcaaggtggtgagcaccgacgagtacgtgaccaggaccaacatctactaccacgccggcagcgccaggctgctgaccgtgggccacccctactacagcatccccaagagcgacaaccccaagaagatcgtggtgcccaaggtgagcggcctgcagtacagggtgttcagggtgaggctgcccgaccccaacaagttcggcttccccgacaccagcttctacaaccccgagacccagaggctggtgtgggcctgcgtgggcctggaggtgggcaggggccagcccctgggcgtgggcatcagcggccaccccctgctgaacaagttcgacgacaccgagaacagcaacaggtacgccggcggccccggcaccgacaacagggagtgcatcagcatggactacaagcagacccagctgtgcctgctgggctgcaagccccccatcggcgagcactggggcaagggcagcccctgcagcaacaacgccatcacccccggcgactgcccccccctggagctgaagaacagcgtgatccaggacggcgacatggtggacaccggcttcggcgccatggacttcaccgccctgcaggacaccaagagcaacgtgcccctggacatctgcaacagcatctgcaagtaccccgactacctgaagatggtggccgagccctacggcgacaccctgttcttctacctgaggagggagcagatgttcgtgaggcacttcttcaacaggagcggcaccgtgggcgagagcgtgcccaccgacctgtacatcaagggcagcggcagcaccgccaccctggccaacagcacctacttccccacccccagcggcagcatggtgaccagcgacgcccagatcttcaacaagccctactggatgcagagggcccagggccacaacaacggcatctgctggggcaaccagctgttcgtgaccgtggtggacaccaccaggagcaccaacatgagcgtgtgcgccgccatcgccaacagcgacaccaccttcaagagcagcaacttcaaggagtacctgaggcacggcgaggagttcgacctgcagttcatcttccagctgtgcaagatcaccctgagcgccgacatcatgacctacatccacagcatgaaccccgccatcctggaggactggaacttcggcctgaccaccccccccagcggcagcctggaggacacctacaggttcgtgaccagccaggccatcacctgccagaagtccgccccccagaagcccaaggaggaccccttcaaggactacgtgttctgggaggtgaacctgaaggagaagttcagcgccgacctggaccagttccccctgggcaggaagttcctgctgcaggccggctacaaagccaagccaaaactgaaaagggctgccccaaccagcaccaggacctcctctgccaagaggaagaaggtgaagaagtaaa

SEQ ID NO: 57 - DNA, 1534 bp, Artificial sequence
  3105 Synthetic HPV31 L1 gene
ctgggtaccatgagcctgtggaggcccagcgaggccaccgtgtacctgccccccgtgcccgtgagcaaggtggtgagcaccgacgagtacgtgaccaggaccaacatctactaccacgccggcagcgccaggctgctgaccgtgggccacccctactacagcatccccaagagcgacaaccccaagaagatcgtggtgcccaaggtgagcggcctgcagtacagggtgttcagggtgaggctgcccgaccccaacaagttcggcttccccgacaccagcttctacaaccccgagacccagaggctggtgtgggcctgcgtgggcctggaggtgggcaggggccagcccctgggcgtgggcatcagcggccaccccctgctgaacaagttcgacgacaccgagaacagcaacaggtacgccggcggccccggcaccgacaacagggagtgcatcagcatggactacaagcagacccagctgtgcctgctgggctgcaagccccccatcggcgagcactggggcaagggcagcccctgcagcaacaacgccatcacccccggcgactgcccccccctggagctgaagaacagcgtgatccaggacggcgacatggtggacaccggcttcggcgccatggacttcaccgccctgcaggacaccaagagcaacgtgcccctggacatctgcaacagcatctgcaagtaccccgactacctgaagatggtggccgagccctacggcgacaccctgttcttctacctgaggagggagcagatgttcgtgaggcacttcttcaacaggagcggcaccgtgggcgagagcgtgcccaccgacctgtacatcaagggcagcggcagcaccgccaccctggccaacagcacctacttccccacccccagcggcagcatggtgaccagcgacgcccagatcttcaacaagccctactggatgcagagggcccagggccacaacaacggcatctgctggggcaaccagctgttcgtgaccgtggtggacaccaccaggagcaccaacatgagcgtgtgcgccgccatcgccaacagcgacaccaccttcaagagcagcaacttcaaggagtacctgaggcacggcgaggagttcgacctgcagttcatcttccagctgtgcaagatcaccctgagcgccgacatcatgacctacatccacagcatgaaccccgccatcctggaggactggaacttcggcctgaccaccccccccagcggcagcctggaggacacctacaggttcgtgaccagccaggccatcacctgccagaagtccgccccccagaagcccaaggaggaccccttcaaggactacgtgttctgggaggtgaacctgaaggagaagttcagcgccgacctggaccagttccccctgggcaggaagttcctgctgcaggccggctacagggccaggcccaagttcaaggccggcaagaggagcgcccccagcgccagcaccaccacccccgccaagaggaagaagaccaagaagtaaactcgagctc

SEQ ID NO: 58 - DNA, 1519 bp, Artificial sequence; identical to SEQ ID NO: 6
  3106 Synthetic HPV33 L1 gene

SEQ ID NO: 59 - DNA, 33 bp, Artificial sequence
  3107 HPV31L1 F1
cttggtaccatgagcctgtggaggcccagcgag

SEQ ID NO: 60 - DNA, 38 bp, Artificial sequence
  3108 HPV31L1 R1
gcttggctttgtagccggcctgcagcaggaacttcctg

SEQ ID NO: 61 - DNA, 1444 bp, Artificial sequence
  3109 HPV31L1 amplified sequence 1
cttggtaccatgagcctgtggaggcccagcgaggccaccgtgtacctgccccccgtgcccgtgagcaaggtggtgagcaccgacgagtacgtgaccaggaccaacatctactaccacgccggcagcgccaggctgctgaccgtgggccacccctactacagcatccccaagagcgacaaccccaagaagatcgtggtgcccaaggtgagcggcctgcagtacagggtgttcagggtgaggctgcccgaccccaacaagttcggcttccccgacaccagcttctacaaccccgagacccagaggctggtgtgggcctgcgtgggcctggaggtgggcaggggccagcccctgggcgtgggcatcagcggccaccccctgctgaacaagttcgacgacaccgagaacagcaacaggtacgccggcggccccggcaccgacaacagggagtgcatcagcatggactacaagcagacccagctgtgcctgctgggctgcaagccccccatcggcgagcactggggcaagggcagcccctgcagcaacaacgccatcacccccggcgactgcccccccctggagctgaagaacagcgtgatccaggacggcgacatggtggacaccggcttcggcgccatggacttcaccgccctgcaggacaccaagagcaacgtgcccctggacatctgcaacagcatctgcaagtaccccgactacctgaagatggtggccgagccctacggcgacaccctgttcttctacctgaggagggagcagatgttcgtgaggcacttcttcaacaggagcggcaccgtgggcgagagcgtgcccaccgacctgtacatcaagggcagcggcagcaccgccaccctggccaacagcacctacttccccacccccagcggcagcatggtgaccagcgacgcccagatcttcaacaagccctactggatgcagagggcccagggccacaacaacggcatctgctggggcaaccagctgttcgtgaccgtggtggacaccaccaggagcaccaacatgagcgtgtgcgccgccatcgccaacagcgacaccaccttcaagagcagcaacttcaaggagtacctgaggcacggcgaggagttcgacctgcagttcatcttccagctgtgcaagatcaccctgagcgccgacatcatgacctacatccacagcatgaaccccgccatcctggaggactggaacttcggcctgaccaccccccccagcggcagcctggaggacacctacaggttcgtgaccagccaggccatcacctgccagaagtccgccccccagaagcccaaggaggaccccttcaaggactacgtgttctgggaggtgaacctgaaggagaagttcagcgccgacctggaccagttccccctgggcaggaagttcctgctgcaggccggctacaaagccaagc

SEQ ID NO: 62 - DNA, 35 bp, Artificial sequence
  3110 HPV31L1 F2
ggccggctacaaagccaagccaaaactgaaaaggg

SEQ ID NO: 63 - DNA, 41 bp, Artificial sequence
  3111 HPV31L1 R2
ctgtctagatttacttcttcaccttcttcctcttggcagag

SEQ ID NO: 64 - DNA, 101 bp, Artificial sequence
  3112 HPV31L1 amplified sequence 2
ggccggctacaaagccaagccaaaactgaaaagggctgccccaaccagcaccaggacctcctctgccaagaggaagaaggtgaagaagtaaatctagacag

SEQ ID NO: 65 - protein, 38 aa, Homo sapiens; identical to SEQ ID NO: 13
  3113 Amino acid sequence of HPV type 59 L1 protein aa 471-508

SEQ ID NO: 66 - protein, 472 aa, Homo sapiens
  3501 Amino acid sequence of HPV type 35 L1 protein aa 1-472
MSLWRSNEATVYLPPVSVSKVVSTDEYVTRTNIYYHAGSSRLLAVGHPYYAIKKQDSNKIAVPKVSGLQYRVFRVKLPDPNKFGFPDTSFYDPASQRLVWACTGVEVGRGQPLGVGISGHPLLNKLDDTENSNKYVGNSGTDNRECISMDYKQTQLCLIGCRPPIGEHWGKGTPCNANQVKAGECPPLELLNTVLQDGDMVDTGFGAMDFTTLQANKSDVPLDICSSICKYPDYLKMVSEPYGDMLFFYLRREQMFVRHLFNRAGTVGETVPADLYIKGTTGTLPSTSYFPTPSGSMVTSDAQIFNKPYWLQRAQGHNNGICWSNQLFVTVVDTTRSTNMSVCSAVSSSDSTYKNDNFKEYLRHGEEYDLQFIFQLCKITLTADVMTYIHSMNPSILEDWNFGLTPPPSGTLEDTYRYVTSQAVTCQKPSAPKPKDDPLKNYTFWEVDLKEKFSADLDQFPLGRKFLLQAGL

SEQ ID NO: 67 - protein, 26 aa, Homo sapiens
  3502 Amino acid sequence of HPV type 33 L1 protein aa 474-499
KAKPKLKRAAPTSTRTSSAKRKKVKK

SEQ ID NO: 68 - protein, 498 aa, Artificial sequence
  3503 Amino acid sequence of chimeric HPV type 35 L1 protein
MSLWRSNEATVYLPPVSVSKVVSTDEYVTRTNIYYHAGSSRLLAVGHPYYAIKKQDSNKIAVPKVSGLQYRVFRVKLPDPNKFGFPDTSFYDPASQRLVWACTGVEVGRGQPLGVGISGHPLLNKLDDTENSNKYVGNSGTDNRECISMDYKQTQLCLIGCRPPIGEHWGKGTPCNANQVKAGECPPLELLNTVLQDGDMVDTGFGAMDFTTLQANKSDVPLDICSSICKYPDYLKMVSEPYGDMLFFYLRREQMFVRHLFNRAGTVGETVPADLYIKGTTGTLPSTSYFPTPSGSMVTSDAQIFNKPYWLQRAQGHNNGICWSNQLFVTVVDTTRSTNMSVCSAVSSSDSTYKNDNFKEYLRHGEEYDLQFIFQLCKITLTADVMTYIHSMNPSILEDWNFGLTPPPSGTLEDTYRYVTSQAVTCQKPSAPKPKDDPLKNYTFWEVDLKEKFSADLDQFPLGRKFLLQAGLKAKPKLKRAAPTSTRTSSAKRKKVKK

SEQ ID NO: 69 - DNA, 1498 bp, Artificial sequence
  3504 Nucleotide sequence of chimeric HPV type 35 L1 protein
atgagtctgtggaggagcaatgaggctacagtctacctgcctcctgtgtctgtgagcaaggtggtgagcacagatgaatatgtgaccaggaccaacatctactaccatgctggctccagcagactgctggctgtgggacacccatactatgccatcaagaagcaggacagcaacaagattgctgtgccaaaggtgtctggactccaatacagggtgttcagggtgaaactgcctgacccaaacaagtttggctttcctgacacctccttctatgaccctgccagccagagactggtgtgggcttgtactggagtggaggtgggcaggggacaaccactgggagtgggcatctctggacacccactgctgaacaaactggatgacacagagaacagcaacaaatatgtgggcaactctggcacagacaacagggagtgtatcagtatggactacaagcagacccaactttgtctgattggctgtagacctccaattggagaacactggggcaagggcacaccatgtaatgccaaccaggtgaaggctggagagtgtcctccattggaactgctgaacacagtgctccaagatggagatatggtggacacaggctttggagctatggacttcaccaccctccaagccaacaagtctgatgtgccactggacatctgttccagcatctgtaaataccctgactacctgaaaatggtgtctgaaccatatggagatatgctgttcttctacctgaggagggaacagatgtttgtgagacacctgttcaacagggctggcacagtgggagagacagtgcctgctgacctctacatcaagggcaccacaggcaccctgccaagcacctcctactttccaacaccatctggcagtatggtgacctctgatgcccagattttcaacaagccatactggctccaaagggctcaaggacacaacaatggcatctgttggagcaaccaactttttgtgacagtggtggacaccaccaggagcaccaatatgagtgtgtgttctgctgtgtcctcctctgacagcacctacaagaatgacaacttcaaggaatacctgagacatggagaggaatatgacctccaattcatcttccaactttgtaagattaccctgacagcagatgtgatgacctacatccacagtatgaacccaagcatcttggaggactggaactttggactgacacctcctccatctggcaccttggaggacacctacagatatgtgaccagccaggctgtgacttgtcagaagccatctgccccaaagccaaaggatgacccactgaaaaactacaccttctgggaggtggacctgaaagagaagttctctgctgacctggaccagtttccactgggcaggaagttcctgctccaagcaggactgaaagccaagccaaaactgaaaagggctgccccaaccagcaccaggacctcctctgccaagaggaagaaggtgaagaagtaaa

SEQ ID NO: 70 - DNA, 1528 bp, Artificial sequence
  3505 Synthetic HPV35 L1 gene
ctgggtaccatgagtctgtggaggagcaatgaggctacagtctacctgcctcctgtgtctgtgagcaaggtggtgagcacagatgaatatgtgaccaggaccaacatctactaccatgctggctccagcagactgctggctgtgggacacccatactatgccatcaagaagcaggacagcaacaagattgctgtgccaaaggtgtctggactccaatacagggtgttcagggtgaaactgcctgacccaaacaagtttggctttcctgacacctccttctatgaccctgccagccagagactggtgtgggcttgtactggagtggaggtgggcaggggacaaccactgggagtgggcatctctggacacccactgctgaacaaactggatgacacagagaacagcaacaaatatgtgggcaactctggcacagacaacagggagtgtatcagtatggactacaagcagacccaactttgtctgattggctgtagacctccaattggagaacactggggcaagggcacaccatgtaatgccaaccaggtgaaggctggagagtgtcctccattggaactgctgaacacagtgctccaagatggagatatggtggacacaggctttggagctatggacttcaccaccctccaagccaacaagtctgatgtgccactggacatctgttccagcatctgtaaataccctgactacctgaaaatggtgtctgaaccatatggagatatgctgttcttctacctgaggagggaacagatgtttgtgagacacctgttcaacagggctggcacagtgggagagacagtgcctgctgacctctacatcaagggcaccacaggcaccctgccaagcacctcctactttccaacaccatctggcagtatggtgacctctgatgcccagattttcaacaagccatactggctccaaagggctcaaggacacaacaatggcatctgttggagcaaccaactttttgtgacagtggtggacaccaccaggagcaccaatatgagtgtgtgttctgctgtgtcctcctctgacagcacctacaagaatgacaacttcaaggaatacctgagacatggagaggaatatgacctccaattcatcttccaactttgtaagattaccctgacagcagatgtgatgacctacatccacagtatgaacccaagcatcttggaggactggaactttggactgacacctcctccatctggcaccttggaggacacctacagatatgtgaccagccaggctgtgacttgtcagaagccatctgccccaaagccaaaggatgacccactgaaaaactacaccttctgggaggtggacctgaaagagaagttctctgctgacctggaccagtttccactgggcaggaagttcctgctccaagcaggactgaaagccagaccaaacttcagactgggcaagagggctgcccctgccagcaccagcaagaagtccagcaccaagaggaggaaggtgaagagctaaactcgagctc

SEQ ID NO: 71 - DNA, 1519 bp, Artificial sequence; identical to SEQ ID NO: 6
  3506 Synthetic HPV33 L1 gene

SEQ ID NO: 72 - DNA, 34 bp, Artificial sequence
  3507 HPV35L1 F1
cttggtaccatgagtctgtggaggagcaatgagg

SEQ ID NO: 73 - DNA, 36 bp, Artificial sequence; identical to SEQ ID NO: 34
  3508 HPV35L1 R1

SEQ ID NO: 74 - DNA, 1435 bp, Artificial sequence
  3509 HPV35L1 amplified sequence 1
cttggtaccatgagtctgtggaggagcaatgaggctacagtctacctgcctcctgtgtctgtgagcaaggtggtgagcacagatgaatatgtgaccaggaccaacatctactaccatgctggctccagcagactgctggctgtgggacacccatactatgccatcaagaagcaggacagcaacaagattgctgtgccaaaggtgtctggactccaatacagggtgttcagggtgaaactgcctgacccaaacaagtttggctttcctgacacctccttctatgaccctgccagccagagactggtgtgggcttgtactggagtggaggtgggcaggggacaaccactgggagtgggcatctctggacacccactgctgaacaaactggatgacacagagaacagcaacaaatatgtgggcaactctggcacagacaacagggagtgtatcagtatggactacaagcagacccaactttgtctgattggctgtagacctccaattggagaacactggggcaagggcacaccatgtaatgccaaccaggtgaaggctggagagtgtcctccattggaactgctgaacacagtgctccaagatggagatatggtggacacaggctttggagctatggacttcaccaccctccaagccaacaagtctgatgtgccactggacatctgttccagcatctgtaaataccctgactacctgaaaatggtgtctgaaccatatggagatatgctgttcttctacctgaggagggaacagatgtttgtgagacacctgttcaacagggctggcacagtgggagagacagtgcctgctgacctctacatcaagggcaccacaggcaccctgccaagcacctcctactttccaacaccatctggcagtatggtgacctctgatgcccagattttcaacaagccatactggctccaaagggctcaaggacacaacaatggcatctgttggagcaaccaactttttgtgacagtggtggacaccaccaggagcaccaatatgagtgtgtgttctgctgtgtcctcctctgacagcacctacaagaatgacaacttcaaggaatacctgagacatggagaggaatatgacctccaattcatcttccaactttgtaagattaccctgacagcagatgtgatgacctacatccacagtatgaacccaagcatcttggaggactggaactttggactgacacctcctccatctggcaccttggaggacacctacagatatgtgaccagccaggctgtgacttgtcagaagccatctgccccaaagccaaaggatgacccactgaaaaactacaccttctgggaggtggacctgaaagagaagttctctgctgacctggaccagtttccactgggcaggaagttcctgctccaagcaggactgaaagccaagc

SEQ ID NO: 75 - DNA, 35 bp, Artificial sequence; identical to SEQ ID NO: 36
  3510 HPV35L1 F2

SEQ ID NO: 76 - DNA, 36 bp, Artificial sequence; identical to SEQ ID NO: 37
  3511 HPV35L1 R2

SEQ ID NO: 77 - DNA, 101 bp, Artificial sequence; identical to SEQ ID NO: 38
  3512 HPV35L1 amplified sequence 2

SEQ ID NO: 78 - protein, 38 aa, Homo sapiens; identical to SEQ ID NO: 13
  3513 Amino acid sequence of HPV type 59 L1 protein aa 471-508

SEQ ID NO: 79 - protein, 469 aa, Homo sapiens
  3901 Amino acid sequence of HPV type 39 L1 protein aa 1-469
MAMWRSSDSMVYLPPPSVAKVVNTDDYVTRTGIYYYAGSSRLLTVGHPYFKVGMNGGRKQDIPKVSAYQYRVFRVTLPDPNKFSIPDASLYNPETQRLVWACVGVEVGRGQPLGVGISGHPLYNRQDDTENSPFSSTTNKDSRDNVSVDYKQTQLCIIGCVPAIGEHWGKGKACKPNNVSTGDCPPLELVNTPIEDGDMIDTGYGAMDFGALQETKSEVPLDICQSICKYPDYLQMSADVYGDSMFFCLRREQLFARHFWNRGGMVGDAIPAQLYIKGTDIRANPGSSVYCPSPSGSMVTSDSQLFNKPYWLHKAQGHNNGICWHNQLFLTVVDTTRSTNFTLSTSIESSIPSTYDPSKFKEYTRHVEEYDLQFIFQLCTVTLTTDVMSYIHTMNSSILDNWNFAVAPPPSASLVDTYRYLQSAAITCQKDAPAPEKKDPYDGLKFWNVDLREKFSLELDQFPLGRKFL

SEQ ID NO: 80 - protein, 38 aa, Homo sapiens; identical to SEQ ID NO: 13
  3902 Amino acid sequence of HPV type 59 L1 protein aa 471-508

SEQ ID NO: 81 - protein, 507 aa, Artificial sequence
  3903 Amino acid sequence of chimeric HPV type 39 L1 protein
MAMWRSSDSMVYLPPPSVAKVVNTDDYVTRTGIYYYAGSSRLLTVGHPYFKVGMNGGRKQDIPKVSAYQYRVFRVTLPDPNKFSIPDASLYNPETQRLVWACVGVEVGRGQPLGVGISGHPLYNRQDDTENSPFSSTTNKDSRDNVSVDYKQTQLCIIGCVPAIGEHWGKGKACKPNNVSTGDCPPLELVNTPIEDGDMIDTGYGAMDFGALQETKSEVPLDICQSICKYPDYLQMSADVYGDSMFFCLRREQLFARHFWNRGGMVGDAIPAQLYIKGTDIRANPGSSVYCPSPSGSMVTSDSQLFNKPYWLHKAQGHNNGICWHNQLFLTVVDTTRSTNFTLSTSIESSIPSTYDPSKFKEYTRHVEEYDLQFIFQLCTVTLTTDVMSYIHTMNSSILDNWNFAVAPPPSASLVDTYRYLQSAAITCQKDAPAPEKKDPYDGLKFWNVDLREKFSLELDQFPLGRKFLLQLGARPKPTIGPRKRAAPAPTSTPSPKRVKRRKSSRK

SEQ ID NO: 82 - DNA, 1525 bp, Artificial sequence
  3904 Nucleotide sequence of chimeric HPV type 39 L1 protein
atggctatgtggaggtcctctgacagtatggtctacctgcctcctccatctgtggctaaggtggtgaacacagatgactatgtgaccaggacaggcatctactactatgctggctccagcagactgctgacagtgggacacccatacttcaaggtggggatgaatggaggcaggaagcaggacatcccaaaggtgtctgcctaccaatacagggtgttcagggtgaccctgcctgacccaaacaagttcagcatccctgatgcctccctctacaaccctgagacccagagactggtgtgggcttgtgtgggagtggaggtgggcaggggacaaccactgggagtgggcatctctggacacccactctacaacagacaggatgacacagagaacagcccattctccagcaccaccaacaaggacagcagggacaatgtgtctgtggactacaagcagacccaactttgtatcattggctgtgtgcctgccattggagaacactggggcaagggcaaggcttgtaagccaaacaatgtgagcacaggagactgtcctccattggaactggtgaacacaccaattgaggatggagatatgattgacacaggctatggagctatggactttggagccctccaagagaccaagtctgaggtgccactggacatctgtcagagcatctgtaaataccctgactacctccaaatgagtgctgatgtctatggagacagtatgttcttctgtctgaggagggaacaactttttgccagacacttctggaacaggggagggatggtgggagatgccatccctgcccaactctacatcaagggcacagacatcagggctaaccctggctcctctgtctactgtccaagcccatctggcagtatggtgacctctgacagccaacttttcaacaagccatactggctgcacaaggctcaaggacacaacaatggcatctgttggcacaaccaacttttcctgacagtggtggacaccaccaggagcaccaacttcaccctgagcaccagcattgagtccagcatcccaagcacctatgacccaagcaagttcaaggaatacaccaggcatgtggaggaatatgacctccaattcatcttccaactttgtactgtgaccctgaccacagatgtgatgagttacatccacacaatgaactccagcatcctggacaactggaactttgctgtggctcctcctccatctgcctccctggtggacacctacagatacctccaatctgctgccatcacttgtcagaaggatgcccctgcccctgagaagaaggacccatatgatggactgaagttctggaatgtggacctgagggagaagttctccttggaactggaccagtttccactgggcaggaagttcctgctccaacttggagccagaccaaagccaaccattggaccaaggaagagggctgcccctgccccaaccagcacaccaagcccaaagagggtgaagaggaggaagtccagcaggaagtaaa

SEQ ID NO: 83 - DNA, 1537 bp, Artificial sequence
  3905 Synthetic HPV39 L1 gene
ctgggtaccatggctatgtggaggtcctctgacagtatggtctacctgcctcctccatctgtggctaaggtggtgaacacagatgactatgtgaccaggacaggcatctactactatgctggctccagcagactgctgacagtgggacacccatacttcaaggtggggatgaatggaggcaggaagcaggacatcccaaaggtgtctgcctaccaatacagggtgttcagggtgaccctgcctgacccaaacaagttcagcatccctgatgcctccctctacaaccctgagacccagagactggtgtgggcttgtgtgggagtggaggtgggcaggggacaaccactgggagtgggcatctctggacacccactctacaacagacaggatgacacagagaacagcccattctccagcaccaccaacaaggacagcagggacaatgtgtctgtggactacaagcagacccaactttgtatcattggctgtgtgcctgccattggagaacactggggcaagggcaaggcttgtaagccaaacaatgtgagcacaggagactgtcctccattggaactggtgaacacaccaattgaggatggagatatgattgacacaggctatggagctatggactttggagccctccaagagaccaagtctgaggtgccactggacatctgtcagagcatctgtaaataccctgactacctccaaatgagtgctgatgtctatggagacagtatgttcttctgtctgaggagggaacaactttttgccagacacttctggaacaggggagggatggtgggagatgccatccctgcccaactctacatcaagggcacagacatcagggctaaccctggctcctctgtctactgtccaagcccatctggcagtatggtgacctctgacagccaacttttcaacaagccatactggctgcacaaggctcaaggacacaacaatggcatctgttggcacaaccaacttttcctgacagtggtggacaccaccaggagcaccaacttcaccctgagcaccagcattgagtccagcatcccaagcacctatgacccaagcaagttcaaggaatacaccaggcatgtggaggaatatgacctccaattcatcttccaactttgtactgtgaccctgaccacagatgtgatgagttacatccacacaatgaactccagcatcctggacaactggaactttgctgtggctcctcctccatctgcctccctggtggacacctacagatacctccaatctgctgccatcacttgtcagaaggatgcccctgcccctgagaagaaggacccatatgatggactgaagttctggaatgtggacctgagggagaagttctccttggaactggaccagtttccactgggcaggaagttcctgctccaagccagggtgaggaggagaccaaccattggaccaaggaagagacctgctgccagcacctcctcctcctctgccaccaaacacaagaggaagagggtgagcaagtaaactcgagctc

SEQ ID NO: 84 - DNA, 1546 bp, Artificial sequence
  3906 Synthetic HPV59 L1 gene
ctgggtaccatggctctgtggaggtcctctgacaacaaggtctacctgcctcctccatctgtggctaaggtggtgagcacagatgaatatgtgaccaggaccagcatcttctaccatgctggctccagcagactgctgacagtgggacacccatacttcaaggtgccaaagggaggcaatggcagacaggatgtgccaaaggtgtctgcctaccaatacagggtgttcagggtgaaactgcctgacccaaacaagtttggactgcctgacaacacagtctatgacccaaacagccagagactggtgtgggcttgtgtgggagtggagattggcaggggacaaccactgggagtgggactgtctggacacccactctacaacaaactggatgacacagagaactctcatgtggcatctgctgtggacaccaaggacaccagggacaatgtgtctgtggactacaagcagacccaactttgtatcattggctgtgtgcctgccattggagaacactggaccaagggcacagcctgtaagccaaccacagtggtccagggagactgtcctccattggaactgataaacacaccaattgaggatggagatatggtggacacaggctatggagctatggacttcaaactgctccaagacaacaagtctgaggtgccactggacatctgtcagagcatctgtaaataccctgactacctccaaatgagtgctgatgcctatggagacagtatgttcttctgtctgaggagggaacaggtgtttgccagacacttctggaacaggtctggcacaatgggagaccaacttcctgagtccctctacatcaagggcacagacatcagggctaaccctggctcctacctctacagcccaagcccatctggctctgtggtgacctctgacagccaacttttcaacaagccatactggctgcacaaggctcaaggactgaacaatggcatctgttggcacaaccaacttttcctgacagtggtggacaccaccaggagcaccaacctgtctgtgtgtgccagcaccacctccagcatcccaaatgtctacacaccaacctccttcaaggaatatgccaggcatgtggaggagtttgacctccaattcatcttccaactttgtaagattaccctgaccacagaggtgatgagttacatccacaatatgaacaccaccatcttggaggactggaactttggagtgacacctcctccaacagcctccctggtggacacctacaggtttgtccagtctgctgctgtgacttgtcagaaggacacagcccctcctgtgaagcaggacccatatgacaaactgaagttctggcctgtggacctgaaagagaggttctctgctgacctggaccagtttccactgggcaggaagttcctgctccaacttggagccagaccaaagccaaccattggaccaaggaagagggctgcccctgccccaaccagcacaccaagcccaaagagggtgaagaggaggaagtccagcaggaagtaaactcgagctc

SEQ ID NO: 85 - DNA, 38 bp, Artificial sequence
  3907 HPV39L1 F1
cttggtaccatggctatgtggaggtcctctgacagtat

SEQ ID NO: 86 - DNA, 38 bp, Artificial sequence
  3908 HPV39L1 R1
tccaagttggagcaggaacttcctgcccagtggaaact

SEQ ID NO: 87 - DNA, 1428 bp, Artificial sequence
  3909 HPV39L1 amplified sequence 1
cttggtaccatggctatgtggaggtcctctgacagtatggtctacctgcctcctccatctgtggctaaggtggtgaacacagatgactatgtgaccaggacaggcatctactactatgctggctccagcagactgctgacagtgggacacccatacttcaaggtggggatgaatggaggcaggaagcaggacatcccaaaggtgtctgcctaccaatacagggtgttcagggtgaccctgcctgacccaaacaagttcagcatccctgatgcctccctctacaaccctgagacccagagactggtgtgggcttgtgtgggagtggaggtgggcaggggacaaccactgggagtgggcatctctggacacccactctacaacagacaggatgacacagagaacagcccattctccagcaccaccaacaaggacagcagggacaatgtgtctgtggactacaagcagacccaactttgtatcattggctgtgtgcctgccattggagaacactggggcaagggcaaggcttgtaagccaaacaatgtgagcacaggagactgtcctccattggaactggtgaacacaccaattgaggatggagatatgattgacacaggctatggagctatggactttggagccctccaagagaccaagtctgaggtgccactggacatctgtcagagcatctgtaaataccctgactacctccaaatgagtgctgatgtctatggagacagtatgttcttctgtctgaggagggaacaactttttgccagacacttctggaacaggggagggatggtgggagatgccatccctgcccaactctacatcaagggcacagacatcagggctaaccctggctcctctgtctactgtccaagcccatctggcagtatggtgacctctgacagccaacttttcaacaagccatactggctgcacaaggctcaaggacacaacaatggcatctgttggcacaaccaacttttcctgacagtggtggacaccaccaggagcaccaacttcaccctgagcaccagcattgagtccagcatcccaagcacctatgacccaagcaagttcaaggaatacaccaggcatgtggaggaatatgacctccaattcatcttccaactttgtactgtgaccctgaccacagatgtgatgagttacatccacacaatgaactccagcatcctggacaactggaactttgctgtggctcctcctccatctgcctccctggtggacacctacagatacctccaatctgctgccatcacttgtcagaaggatgcccctgcccctgagaagaaggacccatatgatggactgaagttctggaatgtggacctgagggagaagttctccttggaactggaccagtttccactgggcaggaagttcctgctccaacttgga

SEQ ID NO: 88 - DNA, 37 bp, Artificial sequence
  3910 HPV39L1 F2
aggaagttcctgctccaacttggagccagaccaaagc

SEQ ID NO: 89 - DNA, 40 bp, Artificial sequence
  3911 HPV39L1 R2
ctgtctagatttacttcctgctggacttcctcctcttcac

SEQ ID NO: 90 - DNA, 139 bp, Artificial sequence
  3912 HPV39L1 amplified sequence 2
aggaagttcctgctccaacttggagccagaccaaagccaaccattggaccaaggaagagggctgcccctgccccaaccagcacaccaagcccaaagagggtgaagaggaggaagtccagcaggaagtaaatctagacag

SEQ ID NO: 91 - protein, 26 aa, Homo sapiens
  3913 Amino acid sequence of HPV type 33 L1 protein aa 474-499
KAKPKLKRAAPTSTRTSSAKRKKVKK

SEQ ID NO: 92 - protein, 478 aa, Homo sapiens
  4501 Amino acid sequence of HPV type 45 L1 protein aa 1-478
MALWRPSDSTVYLPPPSVARVVNTDDYVSRTSIFYHAGSSRLLTVGNPYFRVVPSGAGNKQAVPKVSAYQYRVFRVALPDPNKFGLPDSTIYNPETQRLVWACVGMEIGRGQPLGIGLSGHPFYNKLDDTESAHAATAVITQDVRDNVSVDYKQTQLCILGCVPAIGEHWAKGTLCKPAQLQPGDCPPLELKNTIIEDGDMVDTGYGAMDFSTLQDTKCEVPLDICQSICKYPDYLQMSADPYGDSMFFCLRREQLFARHFWNRAGVMGDTVPTDLYIKGTSANMRETPGSCVYSPSPSGSITTSDSQLFNKPYWLHKAQGHNNGICWHNQLFVTVVDTTRSTNLTLCASTQNPVPNTYDPTKFKHYSRHVEEYDLQFIFQLCTITLTAEVMSYIHSMNSSILENWNFGVPPPPTTSLVDTYRFVQSVAVTCQKDTTPPEKQDPYDKLKFWTVDLKEKFSSDLDQYPLGRKFLVQAGL

SEQ ID NO: 93 - protein, 26 aa, Homo sapiens
  4502 Amino acid sequence of HPV type 33 L1 protein aa 474-499
KAKPKLKRAAPTSTRTSSAKRKKVKK

SEQ ID NO: 94 - protein, 504 aa, Artificial sequence
  4503 Amino acid sequence of chimeric HPV type 45 L1 protein
MALWRPSDSTVYLPPPSVARVVNTDDYVSRTSIFYHAGSSRLLTVGNPYFRVVPSGAGNKQAVPKVSAYQYRVFRVALPDPNKFGLPDSTIYNPETQRLVWACVGMEIGRGQPLGIGLSGHPFYNKLDDTESAHAATAVITQDVRDNVSVDYKQTQLCILGCVPAIGEHWAKGTLCKPAQLQPGDCPPLELKNTIIEDGDMVDTGYGAMDFSTLQDTKCEVPLDICQSICKYPDYLQMSADPYGDSMFFCLRREQLFARHFWNRAGVMGDTVPTDLYIKGTSANMRETPGSCVYSPSPSGSITTSDSQLFNKPYWLHKAQGHNNGICWHNQLFVTVVDTTRSTNLTLCASTQNPVPNTYDPTKFKHYSRHVEEYDLQFIFQLCTITLTAEVMSYIHSMNSSILENWNFGVPPPPTTSLVDTYRFVQSVAVTCQKDTTPPEKQDPYDKLKFWTVDLKEKFSSDLDQYPLGRKFLVQAGLKAKPKLKRAAPTSTRTSSAKRKKVKK

SEQ ID NO: 95 - DNA, 1516 bp, Artificial sequence
  4504 Nucleotide sequence of chimeric HPV type 45 L1 protein
atggctctgtggagaccatctgacagcacagtctacctgcctcctccatctgtggcaagggtggtgaacacagatgactatgtgagcaggaccagcatcttctaccatgctggctccagcagactgctgacagtgggcaacccatacttcagggtggtgccaagtggagcaggcaacaagcaggctgtgccaaaggtgtctgcctaccaatacagggtgttcagggtggctctgcctgacccaaacaagtttggactgcctgacagcaccatctacaaccctgagacccagagactggtgtgggcttgtgtggggatggagattggcaggggacaaccactgggcattggactgtctggacacccattctacaacaaactggatgacacagagtctgcccatgctgccacagcagtgattacccaggatgtgagggacaatgtgtctgtggactacaagcagacccaactttgtatcctgggctgtgtgcctgccattggagaacactgggctaagggcaccctgtgtaagcctgcccaactccaacctggagactgtcctccattggaactgaaaaacaccatcattgaggatggagatatggtggacacaggctatggagctatggacttcagcaccctccaagacaccaagtgtgaggtgccactggacatctgtcagagcatctgtaaataccctgactacctccaaatgagtgctgacccatatggagacagtatgttcttctgtctgaggagggaacaactttttgccagacacttctggaacagggctggagtgatgggagacacagtgccaacagacctctacatcaagggcacctctgccaatatgagggagacacctggctcctgtgtctacagcccaagcccatctggcagcatcaccacctctgacagccaacttttcaacaagccatactggctgcacaaggctcaaggacacaacaatggcatctgttggcacaaccaactttttgtgacagtggtggacaccaccaggagcaccaacctgaccctgtgtgccagcacccagaaccctgtgccaaacacctatgacccaaccaagttcaagcactacagcaggcatgtggaggaatatgacctccaattcatcttccaactttgtaccatcaccctgacagcagaggtgatgagttacatccacagtatgaactccagcatcttggagaactggaactttggagtgcctcctcctccaaccacctccctggtggacacctacaggtttgtccagtctgtggctgtgacttgtcagaaggacaccacacctcctgagaagcaggacccatatgacaaactgaagttctggacagtggacctgaaagagaagttctcctctgacctggaccaatacccactgggcaggaagttcctggtccaggctggactgaaagccaagccaaaactgaaaagggctgccccaaccagcaccaggacctcctctgccaagaggaagaaggtgaagaagtaaa

SEQ ID NO: 96 - DNA, 1552 bp, Artificial sequence
  4505 Synthetic HPV45 L1 gene
ctgggtaccatggctctgtggagaccatctgacagcacagtctacctgcctcctccatctgtggcaagggtggtgaacacagatgactatgtgagcaggaccagcatcttctaccatgctggctccagcagactgctgacagtgggcaacccatacttcagggtggtgccaagtggagcaggcaacaagcaggctgtgccaaaggtgtctgcctaccaatacagggtgttcagggtggctctgcctgacccaaacaagtttggactgcctgacagcaccatctacaaccctgagacccagagactggtgtgggcttgtgtggggatggagattggcaggggacaaccactgggcattggactgtctggacacccattctacaacaaactggatgacacagagtctgcccatgctgccacagcagtgattacccaggatgtgagggacaatgtgtctgtggactacaagcagacccaactttgtatcctgggctgtgtgcctgccattggagaacactgggctaagggcaccctgtgtaagcctgcccaactccaacctggagactgtcctccattggaactgaaaaacaccatcattgaggatggagatatggtggacacaggctatggagctatggacttcagcaccctccaagacaccaagtgtgaggtgccactggacatctgtcagagcatctgtaaataccctgactacctccaaatgagtgctgacccatatggagacagtatgttcttctgtctgaggagggaacaactttttgccagacacttctggaacagggctggagtgatgggagacacagtgccaacagacctctacatcaagggcacctctgccaatatgagggagacacctggctcctgtgtctacagcccaagcccatctggcagcatcaccacctctgacagccaacttttcaacaagccatactggctgcacaaggctcaaggacacaacaatggcatctgttggcacaaccaactttttgtgacagtggtggacaccaccaggagcaccaacctgaccctgtgtgccagcacccagaaccctgtgccaaacacctatgacccaaccaagttcaagcactacagcaggcatgtggaggaatatgacctccaattcatcttccaactttgtaccatcaccctgacagcagaggtgatgagttacatccacagtatgaactccagcatcttggagaactggaactttggagtgcctcctcctccaaccacctccctggtggacacctacaggtttgtccagtctgtggctgtgacttgtcagaaggacaccacacctcctgagaagcaggacccatatgacaaactgaagttctggacagtggacctgaaagagaagttctcctctgacctggaccaatacccactgggcaggaagttcctggtccaggctggactgaggaggagaccaaccattggaccaaggaagagacctgctgccagcaccagcacagccagcagacctgccaagagggtgaggattaggagcaagaagtaaactcgagctc

SEQ ID NO: 97 - DNA, 1519 bp, Artificial sequence; identical to SEQ ID NO: 6
  4506 Synthetic HPV33 L1 gene

SEQ ID NO: 98 - DNA, 33 bp, Artificial sequence
  4507 HPV45L1 F1
cttggtaccatggctctgtggagaccatctgac

SEQ ID NO: 99 - DNA, 32 bp, Artificial sequence
  4508 HPV45L1 R1
gcttggctttcagtccagcctggaccaggaac

SEQ ID NO: 100 - DNA, 1453 bp, Artificial sequence
  4509 HPV45L1 amplified sequence 1
cttggtaccatggctctgtggagaccatctgacagcacagtctacctgcctcctccatctgtggcaagggtggtgaacacagatgactatgtgagcaggaccagcatcttctaccatgctggctccagcagactgctgacagtgggcaacccatacttcagggtggtgccaagtggagcaggcaacaagcaggctgtgccaaaggtgtctgcctaccaatacagggtgttcagggtggctctgcctgacccaaacaagtttggactgcctgacagcaccatctacaaccctgagacccagagactggtgtgggcttgtgtggggatggagattggcaggggacaaccactgggcattggactgtctggacacccattctacaacaaactggatgacacagagtctgcccatgctgccacagcagtgattacccaggatgtgagggacaatgtgtctgtggactacaagcagacccaactttgtatcctgggctgtgtgcctgccattggagaacactgggctaagggcaccctgtgtaagcctgcccaactccaacctggagactgtcctccattggaactgaaaaacaccatcattgaggatggagatatggtggacacaggctatggagctatggacttcagcaccctccaagacaccaagtgtgaggtgccactggacatctgtcagagcatctgtaaataccctgactacctccaaatgagtgctgacccatatggagacagtatgttcttctgtctgaggagggaacaactttttgccagacacttctggaacagggctggagtgatgggagacacagtgccaacagacctctacatcaagggcacctctgccaatatgagggagacacctggctcctgtgtctacagcccaagcccatctggcagcatcaccacctctgacagccaacttttcaacaagccatactggctgcacaaggctcaaggacacaacaatggcatctgttggcacaaccaactttttgtgacagtggtggacaccaccaggagcaccaacctgaccctgtgtgccagcacccagaaccctgtgccaaacacctatgacccaaccaagttcaagcactacagcaggcatgtggaggaatatgacctccaattcatcttccaactttgtaccatcaccctgacagcagaggtgatgagttacatccacagtatgaactccagcatcttggagaactggaactttggagtgcctcctcctccaaccacctccctggtggacacctacaggtttgtccagtctgtggctgtgacttgtcagaaggacaccacacctcctgagaagcaggacccatatgacaaactgaagttctggacagtggacctgaaagagaagttctcctctgacctggaccaatacccactgggcaggaagttcctggtccaggctggactgaaagccaagc

SEQ ID NO: 101 - DNA, 35 bp, Artificial sequence
  4510 HPV45L1 F2
ggctggactgaaagccaagccaaaactgaaaaggg

SEQ ID NO: 102 - DNA, 37 bp, Artificial sequence; identical to SEQ ID NO: 11
  4511 HPV45L1 R2

SEQ ID NO: 103 - DNA, 101 bp, Artificial sequence
  4512 HPV45L1 amplified sequence 2
ggctggactgaaagccaagccaaaactgaaaagggctgccccaaccagcaccaggacctcctctgccaagaggaagaaggtgaagaagtaaatctagacag

SEQ ID NO: 104 - protein, 38 aa, Homo sapiens; identical to SEQ ID NO: 13
  4513 Amino acid sequence of HPV type 59 L1 protein aa 471-508

SEQ ID NO: 105 - protein, 474 aa, Homo sapiens
  5101 Amino acid sequence of HPV type 51 L1 protein aa 1-474
MALWRTNDSKVYLPPAPVSRIVNTEEYITRTGIYYYAGSSRLITLGHPYFPIPKTSTRAAIPKVSAFQYRVFRVQLPDPNKFGLPDPNLYNPDTDRLVWGCVGVEVGRGQPLGVGLSGHPLFNKYDDTENSRIANGNAQQDVRDNTSVDNKQTQLCIIGCAPPIGEHWGIGTTCKNTPVPPGDCPPLELVSSVIQDGDMIDTGFGAMDFAALQATKSDVPLDISQSVCKYPDYLKMSADTYGNSMFFHLRREQIFARHYYNKLVGVGEDIPNDYYIKGSGNGRDPIESYIYSATPSGSMITSDSQIFNKPYWLHRAQGHNNGICWNNQLFITCVDTTRSTNLTISTATAAVSPTFTPSNFKQYIRHGEEYELQFIFQLCKITLTTEVMAYLHTMDPTILEQWNFGLTLPPSASLEDAYRFVRNAATSCQKDTPPQAKPDPLAKYKFWDVDLKERFSLDLDQFALGRKFLLQVGV

SEQ ID NO: 106 - protein, 26 aa, Homo sapiens
  5102 Amino acid sequence of HPV type 33 L1 protein aa 474-499
KAKPKLKRAAPTSTRTSSAKRKKVKK

SEQ ID NO: 107 - protein, 500 aa, Artificial sequence
  5103 Amino acid sequence of chimeric HPV type 51 L1 protein
MALWRTNDSKVYLPPAPVSRIVNTEEYITRTGIYYYAGSSRLITLGHPYFPIPKTSTRAAIPKVSAFQYRVFRVQLPDPNKFGLPDPNLYNPDTDRLVWGCVGVEVGRGQPLGVGLSGHPLFNKYDDTENSRIANGNAQQDVRDNTSVDNKQTQLCIIGCAPPIGEHWGIGTTCKNTPVPPGDCPPLELVSSVIQDGDMIDTGFGAMDFAALQATKSDVPLDISQSVCKYPDYLKMSADTYGNSMFFHLRREQIFARHYYNKLVGVGEDIPNDYYIKGSGNGRDPIESYIYSATPSGSMITSDSQIFNKPYWLHRAQGHNNGICWNNQLFITCVDTTRSTNLTISTATAAVSPTFTPSNFKQYIRHGEEYELQFIFQLCKITLTTEVMAYLHTMDPTILEQWNFGLTLPPSASLEDAYRFVRNAATSCQKDTPPQAKPDPLAKYKFWDVDLKERFSLDLDQFALGRKFLLQVGVKAKPKLKRAAPTSTRTSSAKRKKVKK

SEQ ID NO: 108 - DNA, 1504 bp, Artificial sequence
  5104 Nucleotide sequence of chimeric HPV type 51 L1 protein
atggctctgtggaggaccaatgacagcaaggtctacctgcctcctgcccctgtgagcaggattgtgaacacagaggaatacatcaccaggacaggcatctactactatgctggctccagcagactgattaccctgggacacccatactttccaatcccaaagaccagcaccagggctgccatcccaaaggtgtctgccttccaatacagggtgttcagggtccaacttcctgacccaaacaagtttggactgcctgacccaaacctctacaaccctgacacagacagactggtgtggggctgtgtgggagtggaggtgggcaggggacaaccactgggagtgggactgtctggacacccactgttcaacaaatatgatgacacagagaacagcaggattgccaatggcaatgcccaacaggatgtgagggacaacacctctgtggacaacaagcagacccaactttgtatcattggctgtgcccctccaattggagaacactggggcattggcaccacttgtaagaacacacctgtgcctcctggagactgtcctccattggaactggtgtcctctgtgattcaggatggagatatgattgacacaggctttggagctatggactttgctgccctccaagccaccaagtctgatgtgccactggacatcagccagtctgtgtgtaaataccctgactacctgaaaatgagtgctgacacctatggcaacagtatgttcttccacctgaggagggaacagatttttgccagacactactacaacaaactggtgggagtgggagaggacatcccaaatgactactacatcaagggctctggcaatggcagggacccaattgagtcctacatctactctgccacaccatctggcagtatgattacctctgacagccagattttcaacaagccatactggctgcacagggctcaaggacacaacaatggcatctgttggaacaaccaacttttcatcacttgtgtggacaccaccaggagcaccaacctgaccatcagcacagccacagcagcagtgagcccaaccttcacaccaagcaacttcaagcaatacatcagacatggagaggaatatgaactccaattcatcttccaactttgtaagattaccctgaccacagaggtgatggcttacctgcacacaatggacccaaccatcttggaacagtggaactttggactgaccctgcctccatctgcctccttggaggatgcctacaggtttgtgaggaatgctgccacctcctgtcagaaggacacacctccacaggctaagcctgacccactggctaaatacaagttctgggatgtggacctgaaagagaggttctccctggacctggaccagtttgccctgggcaggaagttcctgctccaagtgggagtcaaagccaagccaaaactgaaaagggctgccccaaccagcaccaggacctcctctgccaagaggaagaaggtgaagaagtaaa

SEQ ID NO: 109 - DNA, 1534 bp, Artificial sequence
  5105 Synthetic HPV51 L1 gene
ctgggtaccatggctctgtggaggaccaatgacagcaaggtctacctgcctcctgcccctgtgagcaggattgtgaacacagaggaatacatcaccaggacaggcatctactactatgctggctccagcagactgattaccctgggacacccatactttccaatcccaaagaccagcaccagggctgccatcccaaaggtgtctgccttccaatacagggtgttcagggtccaacttcctgacccaaacaagtttggactgcctgacccaaacctctacaaccctgacacagacagactggtgtggggctgtgtgggagtggaggtgggcaggggacaaccactgggagtgggactgtctggacacccactgttcaacaaatatgatgacacagagaacagcaggattgccaatggcaatgcccaacaggatgtgagggacaacacctctgtggacaacaagcagacccaactttgtatcattggctgtgcccctccaattggagaacactggggcattggcaccacttgtaagaacacacctgtgcctcctggagactgtcctccattggaactggtgtcctctgtgattcaggatggagatatgattgacacaggctttggagctatggactttgctgccctccaagccaccaagtctgatgtgccactggacatcagccagtctgtgtgtaaataccctgactacctgaaaatgagtgctgacacctatggcaacagtatgttcttccacctgaggagggaacagatttttgccagacactactacaacaaactggtgggagtgggagaggacatcccaaatgactactacatcaagggctctggcaatggcagggacccaattgagtcctacatctactctgccacaccatctggcagtatgattacctctgacagccagattttcaacaagccatactggctgcacagggctcaaggacacaacaatggcatctgttggaacaaccaacttttcatcacttgtgtggacaccaccaggagcaccaacctgaccatcagcacagccacagcagcagtgagcccaaccttcacaccaagcaacttcaagcaatacatcagacatggagaggaatatgaactccaattcatcttccaactttgtaagattaccctgaccacagaggtgatggcttacctgcacacaatggacccaaccatcttggaacagtggaactttggactgaccctgcctccatctgcctccttggaggatgcctacaggtttgtgaggaatgctgccacctcctgtcagaaggacacacctccacaggctaagcctgacccactggctaaatacaagttctgggatgtggacctgaaagagaggttctccctggacctggaccagtttgccctgggcaggaagttcctgctccaagtgggagtccagaggaagccaagacctggactgaaaagacctgcctcctctgcctcctcctcctcctcctcctctgccaagaggaagagggtgaagaagtaaactcgagctc

SEQ ID NO: 110 - DNA, 1519 bp, Artificial sequence; identical to SEQ ID NO: 6
  5106 Synthetic HPV33 L1 gene

SEQ ID NO: 111 - DNA, 34 bp, Artificial sequence
  5107 HPV51L1 F1
cttggtaccatggctctgtggaggaccaatgaca

SEQ ID NO: 112 - DNA, 32 bp, Artificial sequence
  5108 HPV51L1 R1
gcttggctttgactcccacttggagcaggaac

SEQ ID NO: 113 - DNA, 1441 bp, Artificial sequence
  5109 HPV51L1 amplified sequence 1
cttggtaccatggctctgtggaggaccaatgacagcaaggtctacctgcctcctgcccctgtgagcaggattgtgaacacagaggaatacatcaccaggacaggcatctactactatgctggctccagcagactgattaccctgggacacccatactttccaatcccaaagaccagcaccagggctgccatcccaaaggtgtctgccttccaatacagggtgttcagggtccaacttcctgacccaaacaagtttggactgcctgacccaaacctctacaaccctgacacagacagactggtgtggggctgtgtgggagtggaggtgggcaggggacaaccactgggagtgggactgtctggacacccactgttcaacaaatatgatgacacagagaacagcaggattgccaatggcaatgcccaacaggatgtgagggacaacacctctgtggacaacaagcagacccaactttgtatcattggctgtgcccctccaattggagaacactggggcattggcaccacttgtaagaacacacctgtgcctcctggagactgtcctccattggaactggtgtcctctgtgattcaggatggagatatgattgacacaggctttggagctatggactttgctgccctccaagccaccaagtctgatgtgccactggacatcagccagtctgtgtgtaaataccctgactacctgaaaatgagtgctgacacctatggcaacagtatgttcttccacctgaggagggaacagatttttgccagacactactacaacaaactggtgggagtgggagaggacatcccaaatgactactacatcaagggctctggcaatggcagggacccaattgagtcctacatctactctgccacaccatctggcagtatgattacctctgacagccagattttcaacaagccatactggctgcacagggctcaaggacacaacaatggcatctgttggaacaaccaacttttcatcacttgtgtggacaccaccaggagcaccaacctgaccatcagcacagccacagcagcagtgagcccaaccttcacaccaagcaacttcaagcaatacatcagacatggagaggaatatgaactccaattcatcttccaactttgtaagattaccctgaccacagaggtgatggcttacctgcacacaatggacccaaccatcttggaacagtggaactttggactgaccctgcctccatctgcctccttggaggatgcctacaggtttgtgaggaatgctgccacctcctgtcagaaggacacacctccacaggctaagcctgacccactggctaaatacaagttctgggatgtggacctgaaagagaggttctccctggacctggaccagtttgccctgggcaggaagttcctgctccaagtgggagtcaaagccaagc

SEQ ID NO: 114 - DNA, 35 bp, Artificial sequence
  5110 HPV51L1 F2
agtgggagtcaaagccaagccaaaactgaaaaggg

SEQ ID NO: 115 - DNA, 36 bp, Artificial sequence; identical to SEQ ID NO: 37
  5111 HPV51L1 R2

SEQ ID NO: 116 - DNA, 101 bp, Artificial sequence
  5112 HPV51L1 amplified sequence 2
agtgggagtcaaagccaagccaaaactgaaaagggctgccccaaccagcaccaggacctcctctgccaagaggaagaaggtgaagaagtaaatctagacag

SEQ ID NO: 117 - protein, 38 aa, Homo sapiens; identical to SEQ ID NO: 13
  5113 Amino acid sequence of HPV type 59 L1 protein aa 471-508

SEQ ID NO: 118 - protein, 478 aa, Homo sapiens
  5201 Amino acid sequence of HPV type 52 L1 protein aa 1-478
MSVWRPSEATVYLPPVPVSKVVSTDEYVSRTSIYYYAGSSRLLTVGHPYFSIKNTSSGNGKKVLVPKVSGLQYRVFRIKLPDPNKFGFPDTSFYNPETQRLVWACTGLEIGRGQPLGVGISGHPLLNKFDDTETSNKYAGKPGIDNRECLSMDYKQTQLCILGCKPPIGEHWGKGTPCNNNSGNPGDCPPLQLINSVIQDGDMVDTGFGCMDFNTLQASKSDVPIDICSSVCKYPDYLQMASEPYGDSLFFFLRREQMFVRHFFNRAGTLGDPVPGDLYIQGSNSGNTATVQSSAFFPTPSGSMVTSESQLFNKPYWLQRAQGHNNGICWGNQLFVTVVDTTRSTNMTLCAEVKKESTYKNENFKEYLRHGEEFDLQFIFQLCKITLTADVMTYIHKMDATILEDWQFGLTPPPSASLEDTYRFVTSTAITCQKNTPPKGKEDPLKDYMFWEVDLKEKFSADLDQFPLGRKFLLQAGL

SEQ ID NO: 119 - protein, 26 aa, Homo sapiens
  5202 Amino acid sequence of HPV type 33 L1 protein aa 474-499
KAKPKLKRAAPTSTRTSSAKRKKVKK

SEQ ID NO: 120 - protein, 504 aa, Artificial sequence
  5203 Amino acid sequence of chimeric HPV type 52 L1 protein
MSVWRPSEATVYLPPVPVSKVVSTDEYVSRTSIYYYAGSSRLLTVGHPYFSIKNTSSGNGKKVLVPKVSGLQYRVFRIKLPDPNKFGFPDTSFYNPETQRLVWACTGLEIGRGQPLGVGISGHPLLNKFDDTETSNKYAGKPGIDNRECLSMDYKQTQLCILGCKPPIGEHWGKGTPCNNNSGNPGDCPPLQLINSVIQDGDMVDTGFGCMDFNTLQASKSDVPIDICSSVCKYPDYLQMASEPYGDSLFFFLRREQMFVRHFFNRAGTLGDPVPGDLYIQGSNSGNTATVQSSAFFPTPSGSMVTSESQLFNKPYWLQRAQGHNNGICWGNQLFVTVVDTTRSTNMTLCAEVKKESTYKNENFKEYLRHGEEFDLQFIFQLCKITLTADVMTYIHKMDATILEDWQFGLTPPPSASLEDTYRFVTSTAITCQKNTPPKGKEDPLKDYMFWEVDLKEKFSADLDQFPLGRKFLLQAGLKAKPKLKRAAPTSTRTSSAKRKKVKK

SEQ ID NO: 121 - DNA, 1516 bp, Artificial sequence
  5204 Nucleotide sequence of chimeric HPV type 52 L1 protein
atgagcgtgtggaggcccagcgaggccaccgtgtacctgccccccgtgcccgtgagcaaggtggtgagcaccgacgagtacgtgagcaggaccagcatctactactacgccggcagcagcaggctgctgaccgtgggccacccctacttcagcatcaagaacaccagcagcggcaacggcaagaaggtgctggtgcccaaggtgagcggcctgcagtacagggtgttcaggatcaagctgcccgaccccaacaagttcggcttccccgacaccagcttctacaaccccgagacccagaggctggtgtgggcctgcaccggcctggagatcggcaggggccagcccctgggcgtgggcatcagcggccaccccctgctgaacaagttcgacgacaccgagaccagcaacaagtacgccggcaagcccggcatcgacaacagggagtgcctgagcatggactacaagcagacccagctgtgcatcctgggctgcaagccccccatcggcgagcactggggcaagggcaccccctgcaacaacaacagcggcaaccccggcgactgcccccccctgcagctgatcaacagcgtgatccaggacggcgacatggtggacaccggcttcggctgcatggacttcaacaccctgcaggccagcaagagcgacgtgcccatcgacatctgcagcagcgtgtgcaagtaccccgactacctgcagatggccagcgagccctacggcgacagcctgttcttcttcctgaggagggagcagatgttcgtgaggcacttcttcaacagggccggcaccctgggcgaccccgtgcccggcgacctgtacatccagggcagcaacagcggcaacaccgccaccgtgcagagcagcgccttcttccccacccccagcggcagcatggtgaccagcgagagccagctgttcaacaagccctactggctgcagagggcccagggccacaacaacggcatctgctggggcaaccagctgttcgtgaccgtggtggacaccaccaggagcaccaacatgaccctgtgcgccgaggtgaagaaggagagcacctacaagaacgagaacttcaaggagtacctgaggcacggcgaggagttcgacctgcagttcatcttccagctgtgcaagatcaccctgaccgccgacgtgatgacctacatccacaagatggacgccaccatcctggaggactggcagttcggcctgacccccccccccagcgccagcctggaggacacctacaggttcgtgaccagcaccgccatcacctgccagaagaacaccccccccaagggcaaggaggaccccctgaaggactacatgttctgggaggtggacctgaaggagaagttcagcgccgacctggaccagttccccctgggcaggaagttcctgctgcaggccggcctgaaagccaagccaaaactgaaaagggctgccccaaccagcaccaggacctcctctgccaagaggaagaaggtgaagaagtaaa

SEQ ID NO: 122 - DNA, 1531 bp, Artificial sequence
  5205 Synthetic HPV52 L1 gene
ctgggtaccatgagcgtgtggaggcccagcgaggccaccgtgtacctgccccccgtgcccgtgagcaaggtggtgagcaccgacgagtacgtgagcaggaccagcatctactactacgccggcagcagcaggctgctgaccgtgggccacccctacttcagcatcaagaacaccagcagcggcaacggcaagaaggtgctggtgcccaaggtgagcggcctgcagtacagggtgttcaggatcaagctgcccgaccccaacaagttcggcttccccgacaccagcttctacaaccccgagacccagaggctggtgtgggcctgcaccggcctggagatcggcaggggccagcccctgggcgtgggcatcagcggccaccccctgctgaacaagttcgacgacaccgagaccagcaacaagtacgccggcaagcccggcatcgacaacagggagtgcctgagcatggactacaagcagacccagctgtgcatcctgggctgcaagccccccatcggcgagcactggggcaagggcaccccctgcaacaacaacagcggcaaccccggcgactgcccccccctgcagctgatcaacagcgtgatccaggacggcgacatggtggacaccggcttcggctgcatggacttcaacaccctgcaggccagcaagagcgacgtgcccatcgacatctgcagcagcgtgtgcaagtaccccgactacctgcagatggccagcgagccctacggcgacagcctgttcttcttcctgaggagggagcagatgttcgtgaggcacttcttcaacagggccggcaccctgggcgaccccgtgcccggcgacctgtacatccagggcagcaacagcggcaacaccgccaccgtgcagagcagcgccttcttccccacccccagcggcagcatggtgaccagcgagagccagctgttcaacaagccctactggctgcagagggcccagggccacaacaacggcatctgctggggcaaccagctgttcgtgaccgtggtggacaccaccaggagcaccaacatgaccctgtgcgccgaggtgaagaaggagagcacctacaagaacgagaacttcaaggagtacctgaggcacggcgaggagttcgacctgcagttcatcttccagctgtgcaagatcaccctgaccgccgacgtgatgacctacatccacaagatggacgccaccatcctggaggactggcagttcggcctgacccccccccccagcgccagcctggaggacacctacaggttcgtgaccagcaccgccatcacctgccagaagaacaccccccccaagggcaaggaggaccccctgaaggactacatgttctgggaggtggacctgaaggagaagttcagcgccgacctggaccagttccccctgggcaggaagttcctgctgcaggccggcctgcaggccaggcccaagctgaagaggcccgccagcagcgcccccaggaccagcaccaagaagaagaaggtgaagaggtaaactcgagctc

SEQ ID NO: 123 - DNA, 1519 bp, Artificial sequence; identical to SEQ ID NO: 6
  5206 Synthetic HPV33 L1 gene

SEQ ID NO: 124 - DNA, 34 bp, Artificial sequence
  5207 HPV52L1 F1
cttggtaccatgagcgtgtggaggcccagcgagg

SEQ ID NO: 125 - DNA, 35 bp, Artificial sequence
  5208 HPV52L1 R1
gcttggctttcaggccggcctgcagcaggaacttc

SEQ ID NO: 126 - DNA, 1453 bp, Artificial sequence
  5209 HPV52L1 amplified sequence 1
cttggtaccatgagcgtgtggaggcccagcgaggccaccgtgtacctgccccccgtgcccgtgagcaaggtggtgagcaccgacgagtacgtgagcaggaccagcatctactactacgccggcagcagcaggctgctgaccgtgggccacccctacttcagcatcaagaacaccagcagcggcaacggcaagaaggtgctggtgcccaaggtgagcggcctgcagtacagggtgttcaggatcaagctgcccgaccccaacaagttcggcttccccgacaccagcttctacaaccccgagacccagaggctggtgtgggcctgcaccggcctggagatcggcaggggccagcccctgggcgtgggcatcagcggccaccccctgctgaacaagttcgacgacaccgagaccagcaacaagtacgccggcaagcccggcatcgacaacagggagtgcctgagcatggactacaagcagacccagctgtgcatcctgggctgcaagccccccatcggcgagcactggggcaagggcaccccctgcaacaacaacagcggcaaccccggcgactgcccccccctgcagctgatcaacagcgtgatccaggacggcgacatggtggacaccggcttcggctgcatggacttcaacaccctgcaggccagcaagagcgacgtgcccatcgacatctgcagcagcgtgtgcaagtaccccgactacctgcagatggccagcgagccctacggcgacagcctgttcttcttcctgaggagggagcagatgttcgtgaggcacttcttcaacagggccggcaccctgggcgaccccgtgcccggcgacctgtacatccagggcagcaacagcggcaacaccgccaccgtgcagagcagcgccttcttccccacccccagcggcagcatggtgaccagcgagagccagctgttcaacaagccctactggctgcagagggcccagggccacaacaacggcatctgctggggcaaccagctgttcgtgaccgtggtggacaccaccaggagcaccaacatgaccctgtgcgccgaggtgaagaaggagagcacctacaagaacgagaacttcaaggagtacctgaggcacggcgaggagttcgacctgcagttcatcttccagctgtgcaagatcaccctgaccgccgacgtgatgacctacatccacaagatggacgccaccatcctggaggactggcagttcggcctgacccccccccccagcgccagcctggaggacacctacaggttcgtgaccagcaccgccatcacctgccagaagaacaccccccccaagggcaaggaggaccccctgaaggactacatgttctgggaggtggacctgaaggagaagttcagcgccgacctggaccagttccccctgggcaggaagttcctgctgcaggccggcctgaaagccaagc

SEQ ID NO: 127 - DNA, 35 bp, Artificial sequence
  5210 HPV52L1 F2
ggccggcctgaaagccaagccaaaactgaaaaggg

SEQ ID NO: 128 - DNA, 36 bp, Artificial sequence; identical to SEQ ID NO: 37
  5211 HPV52L1 R2

SEQ ID NO: 129 - DNA, 101 bp, Artificial sequence
  5212 HPV52L1 amplified sequence 2
ggccggcctgaaagccaagccaaaactgaaaagggctgccccaaccagcaccaggacctcctctgccaagaggaagaaggtgaagaagtaaatctagacag

SEQ ID NO: 130 - protein, 38 aa, Homo sapiens; identical to SEQ ID NO: 13
  5213 Amino acid sequence of HPV type 59 L1 protein aa 471-508

SEQ ID NO: 131 - protein, 467 aa, Homo sapiens
  5601 Amino acid sequence of HPV type 56 L1 protein aa 1-467
MATWRPSENKVYLPPTPVSKVVATDSYVKRTSIFYHAGSSRLLAVGHPYYSVTKDNTKTNIPKVSAYQYRVFRVRLPDPNKFGLPDTNIYNPDQERLVWACVGLEVGRGQPLGAGLSGHPLFNRLDDTESSNLANNNVIEDSRDNISVDGKQTQLCIVGCTPAMGEHWTKGAVCKSTQVTTGDCPPLALINTPIEDGDMIDTGFGAMDFKVLQESKAEVPLDIVQSTCKYPDYLKMSADAYGDSMWFYLRREQLFARHYFNRAGKVGETIPAELYLKGSNGREPPPSSVYVATPSGSMITSEAQLFNKPYWLQRAQGHNNGICWGNQLFVTVVDTTRSTNMTISTATEQLSKYDARKINQYLRHVEEYELQFVFQLCKITLSAEVMAYLHNMNANLLEDWNIGLSPPVATSLEDKYRYVRSTAITCQREQPPTEKQDPLAKYKFWDVNLQDSFSTDLDQFPLGRKFL

SEQ ID NO: 132 - protein, 31 aa, Homo sapiens
  5602 Amino acid sequence of HPV type 33 L1 protein aa 469-499
LQAGLKAKPKLKRAAPTSTRTSSAKRKKVKK

SEQ ID NO: 133 - protein, 498 aa, Artificial sequence
  5603 Amino acid sequence of chimeric HPV type 56 L1 protein
MATWRPSENKVYLPPTPVSKVVATDSYVKRTSIFYHAGSSRLLAVGHPYYSVTKDNTKTNIPKVSAYQYRVFRVRLPDPNKFGLPDTNIYNPDQERLVWACVGLEVGRGQPLGAGLSGHPLFNRLDDTESSNLANNNVIEDSRDNISVDGKQTQLCIVGCTPAMGEHWTKGAVCKSTQVTTGDCPPLALINTPIEDGDMIDTGFGAMDFKVLQESKAEVPLDIVQSTCKYPDYLKMSADAYGDSMWFYLRREQLFARHYFNRAGKVGETIPAELYLKGSNGREPPPSSVYVATPSGSMITSEAQLFNKPYWLQRAQGHNNGICWGNQLFVTVVDTTRSTNMTISTATEQLSKYDARKINQYLRHVEEYELQFVFQLCKITLSAEVMAYLHNMNANLLEDWNIGLSPPVATSLEDKYRYVRSTAITCQREQPPTEKQDPLAKYKFWDVNLQDSFSTDLDQFPLGRKFLLQAGLKAKPKLKRAAPTSTRTSSAKRKKVKK

SEQ ID NO: 134 - DNA, 1498 bp, Artificial sequence
  5604 Nucleotide sequence of chimeric HPV type 56 L1 protein
atggctacctggagaccatctgagaacaaggtctacctgcctccaacacctgtgagcaaggtggtggctacagactcctatgtgaagaggaccagcatcttctaccatgctggctccagcagactgctggctgtgggacacccatactactctgtgaccaaggacaacaccaagaccaacatcccaaaggtgtctgcctaccaatacagggtgttcagggtgagactgcctgacccaaacaagtttggactgcctgacaccaacatctacaaccctgaccaggagagactggtgtgggcttgtgtgggattggaggtgggcaggggacaaccactgggagcaggactgtctggacacccactgttcaacagactggatgacacagagtccagcaacctggctaacaacaatgtgattgaggacagcagggacaacatctctgtggatggcaagcagacccaactttgtattgtgggctgtactcctgctatgggagaacactggaccaagggagcagtgtgtaagagcacccaggtgaccacaggagactgtcctccactggctctgataaacacaccaattgaggatggagatatgattgacacaggctttggagctatggacttcaaggtgctccaagagagcaaggctgaggtgccactggacattgtccagagcacttgtaaataccctgactacctgaaaatgagtgctgatgcctatggagacagtatgtggttctacctgaggagggaacaactttttgccagacactacttcaacagggctggcaaggtgggagagaccatccctgctgaactctacctgaaaggcagcaatggcagggaacctcctccatcctctgtctatgtggctacaccatctggcagtatgattacctctgaggctcaacttttcaacaagccatactggctccaaagggctcaaggacacaacaatggcatctgttggggcaaccaactttttgtgacagtggtggacaccaccaggagcaccaatatgaccatcagcacagccacagaacaacttagcaaatatgatgccaggaagataaaccaatacctgaggcatgtggaggaatatgaactccaatttgtgttccaactttgtaagattaccctgtctgctgaggtgatggcttacctgcacaatatgaatgccaacctgttggaggactggaacattggactgagccctcctgtggctacctccttggaggacaaatacagatatgtgaggagcacagccatcacttgtcagagggaacaacctccaacagagaagcaggacccactggctaaatacaagttctgggatgtgaacctccaagactccttcagcacagacctggaccagtttccactgggcaggaagttcctgctccaagcaggactgaaagccaagccaaaactgaaaagggctgccccaaccagcaccaggacctcctctgccaagaggaagaaggtgaagaagtaaa

SEQ ID NO: 135 - DNA, 1519 bp, Artificial sequence
  5605 Synthetic HPV56 L1 gene
ctgggtaccatggctacctggagaccatctgagaacaaggtctacctgcctccaacacctgtgagcaaggtggtggctacagactcctatgtgaagaggaccagcatcttctaccatgctggctccagcagactgctggctgtgggacacccatactactctgtgaccaaggacaacaccaagaccaacatcccaaaggtgtctgcctaccaatacagggtgttcagggtgagactgcctgacccaaacaagtttggactgcctgacaccaacatctacaaccctgaccaggagagactggtgtgggcttgtgtgggattggaggtgggcaggggacaaccactgggagcaggactgtctggacacccactgttcaacagactggatgacacagagtccagcaacctggctaacaacaatgtgattgaggacagcagggacaacatctctgtggatggcaagcagacccaactttgtattgtgggctgtactcctgctatgggagaacactggaccaagggagcagtgtgtaagagcacccaggtgaccacaggagactgtcctccactggctctgataaacacaccaattgaggatggagatatgattgacacaggctttggagctatggacttcaaggtgctccaagagagcaaggctgaggtgccactggacattgtccagagcacttgtaaataccctgactacctgaaaatgagtgctgatgcctatggagacagtatgtggttctacctgaggagggaacaactttttgccagacactacttcaacagggctggcaaggtgggagagaccatccctgctgaactctacctgaaaggcagcaatggcagggaacctcctccatcctctgtctatgtggctacaccatctggcagtatgattacctctgaggctcaacttttcaacaagccatactggctccaaagggctcaaggacacaacaatggcatctgttggggcaaccaactttttgtgacagtggtggacaccaccaggagcaccaatatgaccatcagcacagccacagaacaacttagcaaatatgatgccaggaagataaaccaatacctgaggcatgtggaggaatatgaactccaatttgtgttccaactttgtaagattaccctgtctgctgaggtgatggcttacctgcacaatatgaatgccaacctgttggaggactggaacattggactgagccctcctgtggctacctccttggaggacaaatacagatatgtgaggagcacagccatcacttgtcagagggaacaacctccaacagagaagcaggacccactggctaaatacaagttctgggatgtgaacctccaagactccttcagcacagacctggaccagtttccactgggcaggaagttcctgatgcaacttggcaccaggagcaagcctgctgtggctaccagcaagaagaggtctgccccaaccagcaccagcacacctgccaagaggaagaggaggtaaactcgagctc

SEQ ID NO: 136 - DNA, 1519 bp, Artificial sequence; identical to SEQ ID NO: 6
  5606 Synthetic HPV33 L1 gene

SEQ ID NO: 137 - DNA, 33 bp, Artificial sequence
  5607 HPV56L1 F1
cttggtaccatggctacctggagaccatctgag

SEQ ID NO: 138 - DNA, 31 bp, Artificial sequence
  5608 HPV56L1 R1
ctgcttggagcaggaacttcctgcccagtgg

SEQ ID NO: 139 - DNA, 1420 bp, Artificial sequence
  5609 HPV56L1 amplified sequence 1
cttggtaccatggctacctggagaccatctgagaacaaggtctacctgcctccaacacctgtgagcaaggtggtggctacagactcctatgtgaagaggaccagcatcttctaccatgctggctccagcagactgctggctgtgggacacccatactactctgtgaccaaggacaacaccaagaccaacatcccaaaggtgtctgcctaccaatacagggtgttcagggtgagactgcctgacccaaacaagtttggactgcctgacaccaacatctacaaccctgaccaggagagactggtgtgggcttgtgtgggattggaggtgggcaggggacaaccactgggagcaggactgtctggacacccactgttcaacagactggatgacacagagtccagcaacctggctaacaacaatgtgattgaggacagcagggacaacatctctgtggatggcaagcagacccaactttgtattgtgggctgtactcctgctatgggagaacactggaccaagggagcagtgtgtaagagcacccaggtgaccacaggagactgtcctccactggctctgataaacacaccaattgaggatggagatatgattgacacaggctttggagctatggacttcaaggtgctccaagagagcaaggctgaggtgccactggacattgtccagagcacttgtaaataccctgactacctgaaaatgagtgctgatgcctatggagacagtatgtggttctacctgaggagggaacaactttttgccagacactacttcaacagggctggcaaggtgggagagaccatccctgctgaactctacctgaaaggcagcaatggcagggaacctcctccatcctctgtctatgtggctacaccatctggcagtatgattacctctgaggctcaacttttcaacaagccatactggctccaaagggctcaaggacacaacaatggcatctgttggggcaaccaactttttgtgacagtggtggacaccaccaggagcaccaatatgaccatcagcacagccacagaacaacttagcaaatatgatgccaggaagataaaccaatacctgaggcatgtggaggaatatgaactccaatttgtgttccaactttgtaagattaccctgtctgctgaggtgatggcttacctgcacaatatgaatgccaacctgttggaggactggaacattggactgagccctcctgtggctacctccttggaggacaaatacagatatgtgaggagcacagccatcacttgtcagagggaacaacctccaacagagaagcaggacccactggctaaatacaagttctgggatgtgaacctccaagactccttcagcacagacctggaccagtttccactgggcaggaagttcctgctccaagcag

SEQ ID NO: 140 - DNA, 36 bp, Artificial sequence
  5610 HPV56L1 F2
gaagttcctgctccaagcaggactgaaagccaagcc

SEQ ID NO: 141 - DNA, 36 bp, Artificial sequence; identical to SEQ ID NO: 37
  5611 HPV56L1 R2

SEQ ID NO: 142 - DNA, 116 bp, Artificial sequence
  5612 HPV56L1 amplified sequence 2
gaagttcctgctccaagcaggactgaaagccaagccaaaactgaaaagggctgccccaaccagcaccaggacctcctctgccaagaggaagaaggtgaagaagtaaatctagacag

SEQ ID NO: 143 - protein, 38 aa, Homo sapiens; identical to SEQ ID NO: 13
  5613 Amino acid sequence of HPV type 59 L1 protein aa 471-508

SEQ ID NO: 144 - protein, 473 aa, Homo sapiens
  5801 Amino acid sequence of HPV type 58 L1 protein aa 1-473
MSVWRPSEATVYLPPVPVSKVVSTDEYVSRTSIYYYAGSSRLLAVGNPYFSIKSPNNNKKVLVPKVSGLQYRVFRVRLPDPNKFGFPDTSFYNPDTQRLVWACVGLEIGRGQPLGVGVSGHPYLNKFDDTETSNRYPAQPGSDNRECLSMDYKQTQLCLIGCKPPTGEHWGKGVACNNNAAATDCPPLELFNSIIEDGDMVDTGFGCMDFGTLQANKSDVPIDICNSTCKYPDYLKMASEPYGDSLFFFLRREQMFVRHFFNRAGKLGEAVPDDLYIKGSGNTAVIQSSAFFPTPSGSIVTSESQLFNKPYWLQRAQGHNNGICWGNQLFVTVVDTTRSTNMTLCTEVTKEGTYKNDNFKEYVRHVEEYDLQFVFQLCKITLTAEIMTYIHTMDSNILEDWQFGLTPPPSASLQDTYRFVTSQAITCQKTAPPKEKEDPLNKYTFWEVNLKEKFSADLDQFPLGRKFLLQSGL

SEQ ID NO: 145 - protein, 26 aa, Homo sapiens
  5802 Amino acid sequence of HPV type 33 L1 protein aa 474-499
KAKPKLKRAAPTSTRTSSAKRKKVKK

SEQ ID NO: 146 - protein, 499 aa, Artificial sequence
  5803 Amino acid sequence of chimeric HPV type 58 L1 protein
MSVWRPSEATVYLPPVPVSKVVSTDEYVSRTSIYYYAGSSRLLAVGNPYFSIKSPNNNKKVLVPKVSGLQYRVFRVRLPDPNKFGFPDTSFYNPDTQRLVWACVGLEIGRGQPLGVGVSGHPYLNKFDDTETSNRYPAQPGSDNRECLSMDYKQTQLCLIGCKPPTGEHWGKGVACNNNAAATDCPPLELFNSIIEDGDMVDTGFGCMDFGTLQANKSDVPIDICNSTCKYPDYLKMASEPYGDSLFFFLRREQMFVRHFFNRAGKLGEAVPDDLYIKGSGNTAVIQSSAFFPTPSGSIVTSESQLFNKPYWLQRAQGHNNGICWGNQLFVTVVDTTRSTNMTLCTEVTKEGTYKNDNFKEYVRHVEEYDLQFVFQLCKITLTAEIMTYIHTMDSNILEDWQFGLTPPPSASLQDTYRFVTSQAITCQKTAPPKEKEDPLNKYTFWEVNLKEKFSADLDQFPLGRKFLLQSGLKAKPKLKRAAPTSTRTSSAKRKKVKK

SEQ ID NO: 147 - DNA, 1501 bp, Artificial sequence
  5804 Nucleotide sequence of chimeric HPV type 58 L1 protein
atgagcgtgtggaggcccagcgaggccaccgtgtacctgccccccgtgcccgtgagcaaggtggtgagcaccgacgagtacgtgagcaggaccagcatctactactacgccggcagcagcaggctgctggccgtgggcaacccctacttcagcatcaagagccccaacaacaacaagaaggtgctggtgcccaaggtgagcggcctgcagtacagggtgttcagggtgaggctgcccgaccccaacaagttcggcttccccgacaccagcttctacaaccccgacacccagaggctggtgtgggcctgcgtgggcctggagatcggcaggggccagcccctgggcgtgggcgtgagcggccacccctacctgaacaagttcgacgacaccgagaccagcaacaggtaccccgcccagcccggcagcgacaacagggagtgcctgagcatggactacaagcagacccagctgtgcctgatcggctgcaagccccccaccggcgagcactggggcaagggcgtggcctgcaacaacaacgccgccgccaccgactgcccccccctggagctgttcaacagcatcatcgaggacggcgacatggtggacaccggcttcggctgcatggacttcggcaccctgcaggccaacaagagcgacgtgcccatcgacatctgcaacagcacctgcaagtaccccgactacctgaagatggccagcgagccctacggcgacagcctgttcttcttcctgaggagggagcagatgttcgtgaggcacttcttcaacagggccggcaagctgggcgaggccgtgcccgacgacctgtacatcaagggcagcggcaacaccgccgtgatccagagcagcgccttcttccccacccccagcggcagcatcgtgaccagcgagagccagctgttcaacaagccctactggctgcagagggcccagggccacaacaacggcatctgctggggcaaccagctgttcgtgaccgtggtggacaccaccaggagcaccaacatgaccctgtgcaccgaggtgaccaaggagggcacctacaagaacgacaacttcaaggagtacgtgaggcacgtggaggagtacgacctgcagttcgtgttccagctgtgcaagatcaccctgaccgccgagatcatgacctacatccacaccatggacagcaacatcctggaggactggcagttcggcctgacccccccccccagcgccagcctgcaggacacctacaggttcgtgaccagccaggccatcacctgccagaagaccgccccccccaaggagaaggaggaccccctgaacaagtacaccttctgggaggtgaacctgaaggagaagttcagcgccgacctggaccagttccccctgggcaggaagttcctgctgcagagcggcctgaaagccaagccaaaactgaaaagggctgccccaaccagcaccaggacctcctctgccaagaggaagaaggtgaagaagtaaa

SEQ ID NO: 148 - DNA, 1516 bp, Artificial sequence
  5805 Synthetic HPV58 L1 gene
ctgggtaccatgagcgtgtggaggcccagcgaggccaccgtgtacctgccccccgtgcccgtgagcaaggtggtgagcaccgacgagtacgtgagcaggaccagcatctactactacgccggcagcagcaggctgctggccgtgggcaacccctacttcagcatcaagagccccaacaacaacaagaaggtgctggtgcccaaggtgagcggcctgcagtacagggtgttcagggtgaggctgcccgaccccaacaagttcggcttccccgacaccagcttctacaaccccgacacccagaggctggtgtgggcctgcgtgggcctggagatcggcaggggccagcccctgggcgtgggcgtgagcggccacccctacctgaacaagttcgacgacaccgagaccagcaacaggtaccccgcccagcccggcagcgacaacagggagtgcctgagcatggactacaagcagacccagctgtgcctgatcggctgcaagccccccaccggcgagcactggggcaagggcgtggcctgcaacaacaacgccgccgccaccgactgcccccccctggagctgttcaacagcatcatcgaggacggcgacatggtggacaccggcttcggctgcatggacttcggcaccctgcaggccaacaagagcgacgtgcccatcgacatctgcaacagcacctgcaagtaccccgactacctgaagatggccagcgagccctacggcgacagcctgttcttcttcctgaggagggagcagatgttcgtgaggcacttcttcaacagggccggcaagctgggcgaggccgtgcccgacgacctgtacatcaagggcagcggcaacaccgccgtgatccagagcagcgccttcttccccacccccagcggcagcatcgtgaccagcgagagccagctgttcaacaagccctactggctgcagagggcccagggccacaacaacggcatctgctggggcaaccagctgttcgtgaccgtggtggacaccaccaggagcaccaacatgaccctgtgcaccgaggtgaccaaggagggcacctacaagaacgacaacttcaaggagtacgtgaggcacgtggaggagtacgacctgcagttcgtgttccagctgtgcaagatcaccctgaccgccgagatcatgacctacatccacaccatggacagcaacatcctggaggactggcagttcggcctgacccccccccccagcgccagcctgcaggacacctacaggttcgtgaccagccaggccatcacctgccagaagaccgccccccccaaggagaaggaggaccccctgaacaagtacaccttctgggaggtgaacctgaaggagaagttcagcgccgacctggaccagttccccctgggcaggaagttcctgctgcagagcggcctgaaggccaagcccaggctgaagaggagcgcccccaccaccagggcccccagcaccaagaggaagaaggtgaagaagtaaactcgagctc

SEQ ID NO: 149 - DNA, 1519 bp, Artificial sequence; identical to SEQ ID NO: 6
  5806 Synthetic HPV33 L1 gene

SEQ ID NO: 150 - DNA, 34 bp, Artificial sequence; identical to SEQ ID NO: 124
  5807 HPV58L1 F1

SEQ ID NO: 151 - DNA, 36 bp, Artificial sequence
  5808 HPV58L1 R1
gcttggctttcaggccgctctgcagcaggaacttcc

SEQ ID NO: 152 - DNA, 1438 bp, Artificial sequence
  5809 HPV58L1 amplified sequence 1
cttggtaccatgagcgtgtggaggcccagcgaggccaccgtgtacctgccccccgtgcccgtgagcaaggtggtgagcaccgacgagtacgtgagcaggaccagcatctactactacgccggcagcagcaggctgctggccgtgggcaacccctacttcagcatcaagagccccaacaacaacaagaaggtgctggtgcccaaggtgagcggcctgcagtacagggtgttcagggtgaggctgcccgaccccaacaagttcggcttccccgacaccagcttctacaaccccgacacccagaggctggtgtgggcctgcgtgggcctggagatcggcaggggccagcccctgggcgtgggcgtgagcggccacccctacctgaacaagttcgacgacaccgagaccagcaacaggtaccccgcccagcccggcagcgacaacagggagtgcctgagcatggactacaagcagacccagctgtgcctgatcggctgcaagccccccaccggcgagcactggggcaagggcgtggcctgcaacaacaacgccgccgccaccgactgcccccccctggagctgttcaacagcatcatcgaggacggcgacatggtggacaccggcttcggctgcatggacttcggcaccctgcaggccaacaagagcgacgtgcccatcgacatctgcaacagcacctgcaagtaccccgactacctgaagatggccagcgagccctacggcgacagcctgttcttcttcctgaggagggagcagatgttcgtgaggcacttcttcaacagggccggcaagctgggcgaggccgtgcccgacgacctgtacatcaagggcagcggcaacaccgccgtgatccagagcagcgccttcttccccacccccagcggcagcatcgtgaccagcgagagccagctgttcaacaagccctactggctgcagagggcccagggccacaacaacggcatctgctggggcaaccagctgttcgtgaccgtggtggacaccaccaggagcaccaacatgaccctgtgcaccgaggtgaccaaggagggcacctacaagaacgacaacttcaaggagtacgtgaggcacgtggaggagtacgacctgcagttcgtgttccagctgtgcaagatcaccctgaccgccgagatcatgacctacatccacaccatggacagcaacatcctggaggactggcagttcggcctgacccccccccccagcgccagcctgcaggacacctacaggttcgtgaccagccaggccatcacctgccagaagaccgccccccccaaggagaaggaggaccccctgaacaagtacaccttctgggaggtgaacctgaaggagaagttcagcgccgacctggaccagttccccctgggcaggaagttcctgctgcagagcggcctgaaagccaagc

SEQ ID NO: 153 - DNA, 35 bp, Artificial sequence
  5810 HPV58L1 F2
gagcggcctgaaagccaagccaaaactgaaaaggg

SEQ ID NO: 154 - DNA, 36 bp, Artificial sequence; identical to SEQ ID NO: 37
  5811 HPV58L1 R2

SEQ ID NO: 155 - DNA, 101 bp, Artificial sequence
  5812 HPV58L1 amplified sequence 2
gagcggcctgaaagccaagccaaaactgaaaagggctgccccaaccagcaccaggacctcctctgccaagaggaagaaggtgaagaagtaaatctagacag

SEQ ID NO: 156 - protein, 38 aa, Homo sapiens; identical to SEQ ID NO: 13
  5813 Amino acid sequence of HPV type 59 L1 protein aa 471-508